European Patent Application EP 4 803 904 A1, published September 9, 2026. Title: An improved quantitative immunoassay for the detection of autoantibodies to nephrin. Applicant: EUROIMMUN Medizinische Labordiagnostika AG. Application EP. The sequence listing filed with the application follows.

SEQUENCE LISTING (103 sequences)

SEQ ID NO: 1 - protein, 1055 aa, synthetic construct
  source 1..1055: note = consensus sequence
  SITE 15: note = G or E
  SITE 16: note = M or L
  SITE 18: note = T or M
  SITE 28: note = T or A
  SITE 38: note = S or P
  SITE 39: note = E or A
  SITE 41: note = L or M
  SITE 43: note = V or A
  SITE 49: note = V or A
  SITE 50: note = K or E
  SITE 61: note = V or A
  SITE 74: note = N or D
  SITE 75: note = P or R
  SITE 76: note = K or R
  SITE 77: note = I or M
  SITE 91: note = K or R
  SITE 100: note = A or E
  SITE 114: note = G or S
  SITE 128: note = I or V
  SITE 130: note = S or T
  SITE 131: note = I or V
  SITE 134: note = S or P
  SITE 137: note = V or L
  SITE 139: note = Q or L
  SITE 146: note = S or T
  SITE 147: note = T or M
  SITE 163: note = G or P
  SITE 170: note = D or E
  SITE 173: note = F or I
  SITE 175: note = Q or L
  SITE 179: note = T or V
  SITE 180: note = V or I
  SITE 182: note = D or G
  SITE 183: note = V or I
  SITE 185: note = S or A
  SITE 186: note = S or N
  SITE 193: note = E or Q
  SITE 196: note = F or C
  SITE 198: note = T or V
  SITE 202: note = A or V
  SITE 205: note = T or I
  SITE 207: note = Q or R
  SITE 212: note = G or R
  SITE 213: note = Q or K
  SITE 221: note = N or S
  SITE 226: note = T or A
  SITE 228: note = I or L
  SITE 229: note = K or R
  SITE 230: note = A or V
  SITE 232: note = F or V
  SITE 234: note = M or V
  SITE 236: note = I or V
  SITE 238: note = F or C
  SITE 239: note = P or K
  SITE 240: note = P or W
  SITE 241: note = G or absent
  SITE 243: note = P or absent
  SITE 245: note = I or absent
  SITE 247: note = W or R
  SITE 248: note = P or T
  SITE 249: note = G or E
  SITE 251: note = N or D
  SITE 254: note = H or Q
  SITE 259: note = E or Q
  SITE 267: note = A or S
  SITE 273: note = P or L
  SITE 283: note = K or Q
  SITE 287: note = I or T
  SITE 296: note = A or S
  SITE 299: note = H or R
  SITE 307: note = R or W
  SITE 313: note = A or V
  SITE 314: note = R or Q
  SITE 318: note = Q or E
  SITE 319: note = S or A
  SITE 325: note = A or T
  SITE 327: note = T or I
  SITE 328: note = Q or R
  SITE 331: note = S or G
  SITE 332: note = I or V
  SITE 333: note = T or M
  SITE 343: note = V or I
  SITE 344: note = T or I
  SITE 352: note = S or T
  SITE 359: note = L or V
  SITE 360: note = C or S
  SITE 363: note = T or S
  SITE 373: note = R or Q
  SITE 378: note = G or W
  SITE 385: note = D or E
  SITE 386: note = E or D
  SITE 387: note = T or M
  SITE 389: note = M or V
  SITE 393: note = H or Y
  SITE 406: note = V or A
  SITE 407: note = K or R
  SITE 422: note = D or E
  SITE 425: note = S or T
  SITE 432: note = S or T
  SITE 434: note = T or I
  SITE 436: note = N or S
  SITE 451: note = E or V
  SITE 455: note = I or L
  SITE 457: note = T or A
  SITE 459: note = T or N
  SITE 464: note = V or M
  SITE 473: note = E or D
  SITE 481: note = D or A
  SITE 487: note = D or E
  SITE 488: note = P or S
  SITE 491: note = S or P
  SITE 494: note = P or S
  SITE 498: note = Q or H
  SITE 502: note = V or L
  SITE 508: note = T or I
  SITE 514: note = V or I
  SITE 516: note = I or V
  SITE 517: note = I or T
  SITE 520: note = P or S
  SITE 525: note = K or T
  SITE 527: note = S or T
  SITE 538: note = Q or R
  SITE 539: note = L or F
  SITE 540: note = V or A
  SITE 548: note = L or V
  SITE 554: note = S or A
  SITE 555: note = S or T
  SITE 556: note = A or T
  SITE 561: note = D or E
  SITE 568: note = V or I
  SITE 570: note = I or V
  SITE 577: note = N or S
  SITE 580: note = L or W
  SITE 586: note = R or G
  SITE 588: note = D or E
  SITE 594: note = P or A
  SITE 595: note = Q or R
  SITE 600: note = K or R
  SITE 605: note = S or A
  SITE 607: note = S or T
  SITE 609: note = F or L
  SITE 611: note = R or Q
  SITE 613: note = S or T
  SITE 614: note = S or P
  SITE 619: note = H or Q
  SITE 620: note = R or H
  SITE 624: note = R or S
  SITE 631: note = R or Q
  SITE 634: note = V or M
  SITE 636: note = S or A
  SITE 640: note = L or F
  SITE 645: note = P or R
  SITE 654: note = R or L
  SITE 658: note = V or A
  SITE 661: note = Q or K
  SITE 663: note = Q or E
  SITE 664: note = A or V
  SITE 671: note = S or absent
  SITE 672: note = A or absent
  SITE 673: note = N or S
  SITE 681: note = W or G
  SITE 701: note = G or S
  SITE 705: note = Q or H
  SITE 707: note = W or S
  SITE 714: note = D or G
  SITE 716: note = F or L
  SITE 730: note = A or T
  SITE 731: note = L or R
  SITE 732: note = L or V
  SITE 733: note = K or R
  SITE 737: note = H or Q
  SITE 741: note = T or A
  SITE 742: note = I or V
  SITE 744: note = A or V
  SITE 752: note = N or D
  SITE 753: note = V or I
  SITE 759: note = I or L
  SITE 780: note = E or G
  SITE 781: note = D or E
  SITE 784: note = E or D
  SITE 786: note = N or S
  SITE 792: note = K or M
  SITE 795: note = K or R
  SITE 797: note = S or P
  SITE 802: note = R or Q
  SITE 805: note = Q or H
  SITE 807: note = K or E
  SITE 817: note = I or V
  SITE 818: note = V or A
  SITE 825: note = A or P
  SITE 828: note = G or R
  SITE 830: note = V or L
  SITE 836: note = F or Y
  SITE 839: note = Q or H
  SITE 841: note = D or E
  SITE 842: note = H or Q
  SITE 844: note = T or A
  SITE 867: note = G or A
  SITE 871: note = I or V
  SITE 872: note = D or V
  SITE 881: note = P or A
  SITE 885: note = Q or E
  SITE 899: note = V or I
  SITE 907: note = A or T
  SITE 913: note = Q or H
  SITE 919: note = K or T
  SITE 921: note = T or I
  SITE 925: note = A or P
  SITE 931: note = T or I
  SITE 949: note = V or A
  SITE 950: note = V or M
  SITE 953: note = S or T
  SITE 982: note = S or T
  SITE 986: note = L or H
  SITE 987: note = Y or H
  SITE 988: note = M or V
  SITE 991: note = L or V
  SITE 994: note = Q or D
  SITE 1004: note = K or Q
  SITE 1032: note = S or P
  SITE 1038: note = L or P
  SITE 1039: note = D or H
  SITE 1041: note = A or P
  SITE 1042: note = P or S
  SITE 1045: note = T or P
  SITE 1048: note = P or Q
  SITE 1049: note = L or P
XXXXXXXXXXLLLXXXLXXGLXXXXXXXSXPRGFWALXXNXTXVEGXXXXLXCGVXXPGSXVQWAKDGLLLGPXXXXPXFPRYXLEGDXXXGEFHLXIEXCDLSDDAEYECQVXRSEXGPELVSPXVXLXXLVXPKXLXLTPEAGXXVTWVAGQEYXVXCVSXDAKPAPXIXXXXXGXXXXXXSXXVNXGSXXKLXXXEAXXRVXPXSSDNXXLLVCEXSXPALXXPXXXSXTXNXLXXXXXXXXXXXXLXEGXVRAGXXLELXCXXRGGNPXATLQWLKNGXPXSXAWGTEHXXXVAXSXLVMXVXPEDHGXXLSCXXXNSVSXXXXEXXXXLQVTFPPSAXXILGSXSQXENKNVTXXCXXKSSRPRVLLXWWLGXRQLXPXXXXVXDGLXGGHISMSNLTXLXXREDNGLXLTCEAFSXAFXKETFKKXLXLXVKYPAQKLWIEGPPXGQXXRXGXRVRLXCLAIGGNPXPXLXWXKXSRXVXXXRXXQEXRRVXLGSXEKSGSXFSRELXLXXGPXDNXAXFXCKAGQLSASTXXXVQFPPTNXTILANXXXLRPGXALNLTCXSXSSNPPVXLSXDKEGEXLXXVAXXXXXAPFXGSAAXRXVXLXXXXRDHGXXVTCXAHSXXLXETXSXFYRXNVLYXPEFLGEQVXXVTXVEXGXXLLPVSVXXXPAPEAFNXTFRGYRLSPAGGPRHRILSXGALXLXNVTRADXGXYQLHCQNSEGTAEXXXXLDVXYAPXXRXLXDPTEVXXGXSVDXVCTVDANPILPXMFXWERLGXXXEXXXLDDMEXXSXGXTGRLXIXXAXLXQAGAYQCXXDNGVAPXARXLXRLVVRXAPXVXXPXPLXKVAAAGDSTSSATLHCRARXVPNXXFTWXKNGVXLDLXDPRYTEHXYHQGXXHSSLLTIXNVSAAXDYALFXCXATNXLGSDXXNIQLVSISRPDPPXGLKXXSXXPXSVGLEWKPGFDGGLPQXFXIRYEALXXPGFXXXDVXPXXATXFTLTGLXPSTRYRXWLLASNALGDSGLXDKGXQXXXTTPGXXXXXXXXXXXXPTEXPX

SEQ ID NO: 2 - protein, 1055 aa, synthetic construct
  source 1..1055: note = extracellular domain of human nephrin
MALGTTLRASLLLLGLLTEGLAQLAIPASVPRGFWALPENLTVVEGASVELRCGVSTPGSAVQWAKDGLLLGPDPRIPGFPRYRLEGDPARGEFHLHIEACDLSDDAEYECQVGRSEMGPELVSPRVILSILVPPKLLLLTPEAGTMVTWVAGQEYVVNCVSGDAKPAPDITILLSGQTISDISANVNEGSQQKLFTVEATARVTPRSSDNRQLLVCEASSPALEAPIKASFTVNVLFPPGPPVIEWPGLDEGHVRAGQSLELPCVARGGNPLATLQWLKNGQPVSTAWGTEHTQAVARSVLVMTVRPEDHGAQLSCEAHNSVSAGTQEHGITLQVTFPPSAIIILGSASQTENKNVTLSCVSKSSRPRVLLRWWLGWRQLLPMEETVMDGLHGGHISMSNLTFLARREDNGLTLTCEAFSEAFTKETFKKSLILNVKYPAQKLWIEGPPEGQKLRAGTRVRLVCLAIGGNPEPSLMWYKDSRTVTESRLPQESRRVHLGSVEKSGSTFSRELVLVTGPSDNQAKFTCKAGQLSASTQLAVQFPPTNVTILANASALRPGDALNLTCVSVSSNPPVNLSWDKEGERLEGVAAPPRRAPFKGSAAARSVLLQVSSRDHGQRVTCRAHSAELRETVSSFYRLNVLYRPEFLGEQVLVVTAVEQGEALLPVSVSANPAPEAFNWTFRGYRLSPAGGPRHRILSSGALHLWNVTRADDGLYQLHCQNSEGTAEARLRLDVHYAPTIRALQDPTEVNVGGSVDIVCTVDANPILPGMFNWERLGEDEEDQSLDDMEKISRGPTGRLRIHHAKLAQAGAYQCIVDNGVAPPARRLLRLVVRFAPQVEHPTPLTKVAAAGDSTSSATLHCRARGVPNIVFTWTKNGVPLDLQDPRYTEHTYHQGGVHSSLLTIANVSAAQDYALFTCTATNALGSDQTNIQLVSISRPDPPSGLKVVSLTPHSVGLEWKPGFDGGLPQRFCIRYEALGTPGFHYVDVVPPQATTFTLTGLQPSTRYRVWLLASNALGDSGLADKGTQLPITTPGLHQPSGEPEDQLPTEPPS

SEQ ID NO: 3 - protein, 1078 aa, synthetic construct
  source 1..1078: note = extracellular domain of murine nephrin
MGAKEATVRGPGASPVHRTCHLIPLLLAGMLTTGLAQSPVPTSAPRGFWALSENLTVVEGSTVKLWCGVRAPGSVVQWAKDGLLLGPNPKIPGFPRYSLEGDSAKGEFHLLIEACDLSDDAEYECQVGRSELGPELVSPSVILSILVSPKVLQLTPEAGSTVTWVAGQEYVVTCVSGDAKPAPDIIFIQGGRTVEDVSSSVNEGSEEKLFFTEAEARVTPQSSDNGQLLVCEGSNPALATPIKASFTMNILFPPGPPVIDWPGLNEGHVRAGENLELPCIARGGNPPATLQWLKNGKPVSIAWGTEHAQAVAHSVLVMTVRPEDHGARLSCQSYNSVSAETQERSITLQVTFPPSAVTILGSTSQSENKNVTLCCLTKSSRPRVLLRWWLGGRQLLPTDETVMDGLHGGHISMSNLTLLVKREDNGLSLTCEAFSDAFSKETFKKSLTLNVKYPAQKLWIEGPPEGQSIRTGTRVRLVCLAIGGNPEPSLTWLKDSRPVNDPRQSQEPRRVQLGSVEKSGSTFSRELVLIIGPPDNLAKFSCKAGQLSASTQLVVQFPPTNLTILANSSALRPGDALNLTCVSISSNPPVNLSLDKEGERLDDVAAKPQSAPFKGSAASRSVFLRVSSRDHGHRVTCRAHSEALRETVSSFYRLNVLYPPEFLGEQVRAVTVVEQGQALLPVSVSANPAPEAFNWTFRGYRLSPAGGPRHRILSGGALQLWNVTRADDGFYQLHCQNSEGTAEALLKLDVHYAPTIRALKDPTEVNVGGSVDIVCTVDANPILPEMFSWERLGEDEEELNLDDMEKMSKGSTGRLRIRQAKLSQAGAYQCIVDNGVAPAARGLVRLVVRFAPQVDHPTPLTKVAAAGDSTSSATLHCRARGVPNIDFTWTKNGVPLDLQDPRYTEHKYHQGVVHSSLLTIANVSAAQDYALFKCTATNALGSDHTNIQLVSISRPDPPLGLKVVSVSPHSVGLEWKPGFDGGLPQRFQIRYEALESPGFLYMDVLPAQATTFTLTGLKPSTRYRIWLLASNALGDSGLTDKGIQVSITTPGLDQAPEDTDQPLPTEQPPGPPRLPLLP

SEQ ID NO: 4 - protein, 1078 aa, synthetic construct
  source 1..1078: note = extracellular domain of rat nephrin
MGAKRVTVRGARTSPIHRMSSLTPLLLMGMLTSGLAESPVPTSAPRGFWALSENLTAVEGTTVKLWCGVRAPGSVVQWAKDGLLLGPNPKMPGFPRYSLEGDRAKGEFHLLIEACDLSDDAEYECQVGRSELGPELVSPKVILSILVSPKVLLLTPEAGSTVTWVAGQEYVVTCVSGDAKPAPDITFIQSGRTILDVSSNVNEGSEEKLCITEAEARVIPQSSDNGQLLVCEGSNPALDTPIKASFTMNILFPPGPPVIDWPGLNEGHVRAGENLELPCTARGGNPPATLQWLKNGKPVSTAWGTEHAQAVAHSVLVMTVRPEDHGARLSCQSYNSVSAGTQERSITLQVTFPPSAITILGSVSQSENKNVTLCCLTKSSRPRVLLRWWLGGRQLLPTDETVMDGLHGGHISMSNLTFLVRREDNGLPLTCEAFSDAFSKETFKKSLTLNVKYPAQKLWIEGPPEGQYIRTGTRVRLVCLAIGGNPDPSLIWFKDSRPVSEPRQPQEPRRVQLGSVEKSGSTFSRELVLIIGPPDNRAKFSCKAGQLSASTQLVVQFPPTNLTILANSSALRPGDALNLTCVSISSNPPVNLSWDKEGERLEDVAAKPQSAPFKGSAASRSVFLRVSSRDHGQRVTCRAHSEALRETVSSFYRFNVLYPPEFLGEQVRAVTVVEQGQVLLPVSVSANPAPEAFNWTFRGYRLSPAGGPRHRILSGGALQLWNVTRADDGFYQLHCQNSEGTAEALLKLDVHYAPTIRALRDPTEVNVGGSVDIVCTVDANPILPEMFSWERLGEEEEDLNLDDMEKVSKGSTGRLRIRQAKLSQAGAYQCIVDNGVAPAARGLVRLVVRFAPQVDQPTPLTKVAAAGDSTSSATLHCRARGVPNIDFTWTKNGVPLDLQDPRYTEHRYHQGVVHSSLLTIANVSAAQDYALFKCTATNALGSDHTNIQLVSISRPDPPLGLKVVSISPHSVGLEWKPGFDGGLPQRFQIRYEALETPGFLHVDVLPTQATTFTLTGLKPSTRYRIWLLASNALGDSGLTDKGIQVSVTTPGPDQAPEDTDHQLPTELPPGPPRLPLLP

SEQ ID NO: 5 - protein, 1070 aa, synthetic construct
  source 1..1070: note = extracellular domain of rabbit nephrin
MTEPPRGLEVALRTPIGDALLLMGLLTTGLVQSSVPASAPRGFWALPANLTAVEGAEAELQCGVSAPGSAVQWAKDGLLLGPDPRIPGFPRYRLEGDPAKGEFHLHIEACDLSDDAEYECQVGRSEMGPELVSPRVVLSILVPPKVLQLTPEAGSTVTWVAGQEYVVSCVSPDAKPAPEITFLQSGQTVSDISANVNDGSQEKLFTTEATARVIPQSSDNGQLLVCESSSPALDTPLRASVTMNVLFPPGAPVIEWPGLNEGHVRAGQSLELPCVARGGNPPATLQWLKNGQPLSTAWGTEHVQAVARSVLVMTVWPEDHGARLSCEASNSVSAGTREQSVTLQVTFPPSAITILGSASQSENKNVTLSCITKSSRPRVLLQWWLGGRQLLPTEETVMDGLHGGHISMSNLTYLVRREDNGLTLTCEAFSEAFTKETFKKSLTLSVKYPAQKLWIEGPPEGQLLRTGTRVRLMCLAIGGNPDPALTWLKDSRTVTEPRLPQEPRRVQLGSLEKSGSTFSRELVLVIGPSDNKATFTCKAGQLSASTRLVVQFPPTNLTILANASALRPGDALNLTCISISSNPPVNLSWDKEGEGLESVAGLPQKAPFKGSAAARSVFLRVTSRDHGHHVTCRAHSAELRETVSSFYRLNVLYPPEFLGEQVLEVTAVEQGEALLPVSVSANPAPEAFNWTFRGYRLSPAGGPRHRILSSGALQLWNVTRADGGLYQLHCQNSEGTAEALVRLDVHYAPIIRALQDPTEVDVGGSVDLVCTVDANPILPDMFSWERLGEEEEDQSLDDMEKISKGSTGRLRILHAELAQAGAYQCVVDNGVAPPARGLVRLVVRYAPQVEHPAPLTKVAAAGDSTSSATLHCRARAVPNVVFTWTKNGVPLDLQDPRYTEHTYHQGGVHSSLLTIANVSAAHDYALFTCTATNPLGSDQTNIQLVSISRPDPPSGLKVVSLTPHSVGLEWKPGFDGGLPQKFRIRYEALDTPGFLYMDVLPAQATAFTLTGLQPSTRYRLWLLASNALGDSGLADKGIQLSLTTPGLDHPSGIPDHQPPTEQPAGPPGLR

SEQ ID NO: 6 - protein, 1061 aa, synthetic construct
  source 1..1061: note = extracellular domain of dog nephrin
MALRTPSRAPLLLMGLLTTGLAQLPLSASAPRGFWALPENLTVVEGATAELQCGVHAPGSVVQWAKDGLLLGPDPRIPRFPRYRLEGDPSRGEFHLHIEACDLSDDAEYECQVGRSETGPELVSPRVILSVLVPPKVLQLTPEAGSTVTWVAGQEYVVTCVSGDAKPAPDITFFQSGQTVSDISANVNAGSQEKLFTTEATARVTPQSSDNGQLLVCEGSSPALDTPIRVSVTMNVLFPPGPPVIEWPGLDEGHVRAGQSLELLCVARGGNPPATLQWLKNGQPMSTAWGTEHAEAVARSMLVMVVRPEDHGARLSCEAHNSVSTGIQERGVTLQVTFPPSAITILGSASQSENKNVTLSCISKSSRPRVLLRWWLGWRQLVPTEEMVVDGLHGGHISMSNLTFLVRREDNGLTLTCEAFSEAFTKETFKKSLTLNVKYPAQKLWIEGPPEGQRLRAGTRVRLVCLAIGGNPEPSLTWLKDSRTVTEPRPPQEPRRVQLGSLEKSGSTFSRELILITGPSDNQAKFTCKAGQLSASTQLVVQFPPTNVTILANATALRPGDALNLTCISVSSNPPVNLSWDKEGERLESVATPPRSAPFKGSAAARSVLLRMSSRDHGHRVTCRAHSPELRETMSAFYRLNVLYPPEFLGEQVLVVTAVEQGEALLPVSVSANPAPEAFNWTFRGYRLSPAGGPRHRILSGGALQLWNVTRADDGLYQLHCQNSEGTAETLVRLDVHYAPTIRALQDPTEVNIGGSVDIVCTVDANPILPEMFSWERLGEEEEDQSLDDMEKISKGSTGRLRIHHAKLAQAGAYQCIVDNGVAPPARGLVRLVVRFAPQVEHPTPLNKVAAAGDSTSSATLHCRARGVPNIVFTWAKNGVPLDLEDPRYTEHTYHQGGVHSSLLTIANVSAAQDYALFTCTATNPLGSDHTNIQLVSISRPDPPTGLKVVSMTPYSVGLEWKPGFDGGLPQKFQIRYEALGTPGFLYMDVLPPDATTFTLTGLQPSTRYRVWLLASNALGDSGLTDKGSQIPITTPGLDEPSGEPDYQLPTEQPVGPSGLP

SEQ ID NO: 7 - protein, 1055 aa, synthetic construct
  source 1..1055: note = extracellular domain of cat nephrin
MALRTPGRVPLLLLGLLTTGLARLPLPASTPRGFWALPENLTVVEGATAELRCGVSAPGSAVQWAKDGLLLGPDPRIPSFPRYRLEGDPDRGEFHLHIEACDLSDDAEYECQVGRSETGPELVSPRVILTILVPPKVLQLTPEAGSTVTWVAGQEYVVSCVSGDAKPAPDITFIQSGQTISDISANVNVGSQEKLFTTEATARVTPQSSDNGKLLVCEGSSPALDTPIRVSVTMNVLFPPGPPVIEWPGLDEGHVRAGQSLELLCVSRGGNPPATLQWLKNGQPVSTAWGTEHAEAVARSMLVMIVRPEDHGARLSCEAHNSVSTGIQERGVTLQVTFPPSAITILGSASQSENKNVTLSCITKSSRPRVLLRWWLGWRQLLPTEDMVMDGLHGGHISMSNLTFLVRREDNGLTLTCEAFSEAFTKETFKKSLILNVKYPAQKLWIEGPPEGQRLRAGTRVRLVCLAIGGNPDPSLTWFKDSRAVTEPRPPQEPRRVQLGSLEKSGSTFSRELVLITGPSDNQAKFTCKAGQLSASTQLVVQFPPTNVTILANASALRPGDALNLTCVSVSSNPPVNLSWDKEGERLESVAIPPRSAPFKGSAAARSVLLRMSSRDHGHRVTCRAHSTELRETMSAFYRLNVLYPPEFLGEQVLVVTAVEQGEALLPVSVSANPAPEAFNWTFRGYRLSPAGGPRHRILSGGALQLWNVTRADDGLYQLHCQNSEGTAEALVRLDVHYAPTIRVLQDPTEVNIGGSVDIVCTVDANPILPGMFNWERLGGEEEDHSLDDMEKMSKGSTGRLRIHHAKLDQAGAYQCIVDNGVAPPARGLVRLVVRFAPQVEHPTPLTKVAAAGDSTSSATLHCRARGVPNIVFTWTKNGVALDLQDPRYTEHTYHQGMVHSSLLTIANVSAAQDYALFTCTATNPLGSDRTNIQLVSISRPDPPTGLKVMSMTPYSVGLEWKPGFDGGLPQRFQIRYEALGTPGFLYMDVLPPQATTFTLTGLQPSTRYRVWLLASNALGDSGLMDKGSQISVTTPGLDQPSGEPDYQLPTEQPT

SEQ ID NO: 8 - protein, 1127 aa, synthetic construct
  source 1..1127: note = extracellular domain of equine nephrin
MEGERDRKAERERDLGEERKTEREEMERKRQREKLETDIERGTKRQTEADAGGRQWALGATGRGHGMALRIPVNAPLLLMGLLTTGLAQLPIPASAPRGFWALPENMTVVEGAAAELRCGVSAPGSAVQWAKDGLLLGPDRRIPGFPRYRLEGDPARGEFHLHIEACDLSDDAEYECQVSRSETGPELVSPRVILSVLVPPKVLQLTPEAGSTVTWVAGQEYEVSCVSGDAKPAPDITFVQSGQVIPDISANVNAGSQEKLFTTEAKVRVTPQSSDNGQLLVCEGSSPALDTPIKVSVTMNVLFPPGPPVIEWPGLDEGHVRAGQTLELLCMSRGGNPPATLQWLKNGQPLSTAWGTEHAHSVARSMLVMMVRPEDHGARLSCEAHNSVSTKIQERGVMLQVTFPPSAITILGSASQSENKNVTLSCITKSSRPRVLLRWWLGWRQLQPTEETVMDGLHGGHISMSNLTFLVRREDNGLTLTCEAFSDAFTKETFKKTLTLNVKYPAQKLWIEGPPVGQRLRAGTRVRLVCLAIGGNPDPTLTWYKDSRTVTEPRPPQEPRRVQLGSLEKSGSTFSRELVLVTGPSDNQAKFTCKAGQLSASTQFVVQFPPTNVTILANASALRPGEALNLTCVSVSSNPPVNLSWDKEGERLEGVAARARSAPFRGSAAARSVLLRMSSRDHGHRVTCRAHSAELRETVSAFYRLNVLYPPEFLGEQVLVVTAVEQGEALLPVSVSANPAPEAFNWTFRGYRLSPAGGPRHRILSGGALQLWNVTRADDGLYQLHCQNSEGTAEALVRLDVHYAPAIRALQDPTEVNVGGSVDIVCTVDANPILPGMFQWERLGEEEEDRSLDDMEMTSKGSTGRLQIRQAKLTQAGAYQCIADNGVAPPARGLVRLVVRFAPQVEHPTPLSKVAAAGDSTSSATLHCRARGVPNVVFTWTKNGVPLDLQDPRYTEHTYHQGGVHSSLLTIANVSAAQDYALFTCTATNPLGSDHINIQLVSISRPDPPSGLKVVSMTPYSVGLEWKPGFDGGLPQRFQIRYEALGTPGFLYVDVLPPQATTFTLTGLQPSTRYRVWLLASNALGDSGLADKGSQIPITTPGLDQPSGEPDYQLPTEQPAGPSELP

SEQ ID NO: 9 - protein, 1074 aa, synthetic construct
  source 1..1074: note = extracellular domain of sheep nephrin
EVGANTADIKDRGPGMALSTRIKAELLLLGLLTTGLTQVPILASAPRGFWALPENLTVVEGAVAELRCGVHAPGSAVQWAKDGLLLGPDPRIPSFPRYRLEGDHAKGEFHLRIEACDLSDDAEYECQVGRSETGPELVSPRVILSILVPPKVLQLTPEAGSTVTWVAGQEYTVSCVSGDAKPAPDITFLLSGQTISGISANVNEGSQQKLFTTEATARVTPQSSDNGQLLVCEGSSPALDTPIKASVTMNVLFPPGPPIIEWPGLDEGQVRAGQSLELSCTARGGNPLATLQWLKNGQPVSTAWGTEHAQAVARSLLVMIVRPEDHGARLSCEAYNSVSTGIQERGVTLQVTFPPSAITILGSASQSENKNVTVSCITKSSRPRVLLRWWLGWRQLQPSEETVMDGLHGGHISMSNLTFLARREDNGLTLTCEAFSEAFTKETFKKSLTLNVKYPAQKLWIEGPPEGQRLRAGNRVRLVCLAIGGNPDPSLTWYKASRTVTDPRPPQEPRRVQLGSVEKSGSIFSRELVLITGPSDNQAKFTCKAGQLSASTQLVVQFPPTNVTILANASTLRPGDALNLTCVSVSSNPPVNLSWDKEGERLEGVAAQPRRAPFKGSAAARSVLLRLSSRDHGHRVTCSAHSTELRETVSAFYRLNVLYPPEFLGEQVLVVTAVEQGEALLPVSVSPAPEAFNGTFRGYRLSPAGGPRHRILSGGALQLSNVTRADDGLYQLHCQNSEGTAEALVRLDVQYAPTIRALQDPTEVNVGDSVDIVCTVDANPILPEMFSWERLGEEGEDQSLDDMEKMSKGSTGRLRIHHAKLTQAGAYQCIVDNGVAPPARGLVRLVVRFAPHVEHPAPLTKVAAAGDSTSSATLHCRARGVPNIVFTWTKNGVPLDLQDPRYTEHTYHQGGVHSSLLTIANVSAAQDYALFTCIATNPLGSDHTNIQLVSISRPDPPSGLKAVSVTPYSVGLEWKPGFDGGLPQRFQIRYEALGTPGFLYMDVLPPQATSFTLTGLQPSTRYRVWLLASNALGDSGLVDKGSQISITTPGLDQPSREPDSQLPTEQPAGPSEMP

SEQ ID NO: 10 - protein, 1055 aa, synthetic construct
  source 1..1055: note = extracellular domain of goat nephrin
MALSTRIKAELLLLGLLTTGLTQVPILASAPRGFWALPENLTVVEGAIAELRCGVHAPGSAVQWAKDGLLLGPDPRIPSFPRYRLEGDPAKGEFHLHIEACDLSDDAEYECQVGRSETGPELVSPRVILSILVPPKVLQLTPEAGSTVTWVAGQEYTVSCVSGDAKPAPDITFLLSGQTISGISANVNEGSQQKLFTTEATARVTPQSSDNGQLLVCEGSSPALDTPIKASVTMNVLCKWRTELDEGQVRAGQSLELSCTARGGNPLATLQWLKNGQPVSTAWGTEHAQAVARSLLVMIVRPEDHGVRLSCEAYNSVSTGIQEHGVTLQVTFPPSAITILGSASQSENKNVTVSCITKSSRPRVLLRWWLGWRQLQPSEETVMDGLHGGHISMSNLTFLARREDNGLTLTCEAFSEAFTKETFKKSLTLNVKYPAQKLWIEGPPEGQRLRAGNRVRLVCLAIGGNPDPSLTWYKDSRTVTEPRPPQEPRRVQLGSVEKSGSIFSRELVLITGPSDNQAKFTCKAGQLSASTQLVVQFPPTNVTILANASTLRPGDALNLTCVSVSSNPPVNLSWDKEGERLEGVAAQPRRAPFKGSAAARSVLLRLSSRDHGHRVTCSAHSTELRETVSAFYRLNVLYPPEFLGEQVLVVTAVEQGEALLPVSVSANPAPEAFNWTFRGYRLSPAGGPRHRILSGGALQLWNVTRADDGLYQLHCQNSEGTAEALVRLDVQYAPTVRALQDPTEVNVGASVDIVCTVDANPILPEMFTWERLGEEGEDQSLDDMEKMSKGSTGRLRIHHAKLTQAGAYQCIVDNGVAPPARGLVRLVVRFAPHVEHPAPLTKVAAAGDSTSSATLHCRARGVPNIVFTWTKNGVPLDLQDPRYTEHTYHQGGVHSSLLTITNVSAAQDYALFTCIATNPLGSDHTNIQLVSISRPDPPSGLKAVSMTPYSVGLEWKPGFDGGLPQRFQIRYEALGTPGFLYMDVLPPQATTFTLTGLQPSTRYRVWLLASNALGDSGLVDKGSQISITTPGLDQPSREPDYQLPTEQPAGPSEMP

SEQ ID NO: 11 - protein, 1092 aa, synthetic construct
  source 1..1092: note = extracellular domain of camel nephrin
MRPRERDPERGRGRNRRQEVGPEGATGRGPGMAPRIPIMAPLLLMELLMTGLAQVPIPASAPRGFWALPENLTVVEGAAAELRCGVSSPGSAVQWAKDGLLLGPDPRIPGFPRYHLEGDPTRGEFHLRIEECDLSDDAEYECQVGRSETGPELVSPRVILSVLVPPKVLQLTPEAGSTVTWVAGQEYTVSCVSGDAKPAPDIAFLQRGKTISDISANVNEGSREKLFTTEATARVTPQSSDNGQLLVCEASSPALETPIKVSVTMNILFPPGPPVIEWPGLDEGHVRAGQSLELLCTARGGNPPATLQWLKNGQPVSTAWGTEHAQAVARSLLVMIVRPEDHGARLSCEAHNSVSTGIQERGVTLQVTFPPSAVTILGSASQSENKNVTLSCITKSSRPRVLLRWWLGWRQLLPTEETVMDGLYGGHISMSNLTFLARREDNGLTLTCEAFSEAFTKETFKKSLTLNVKYPAQKLWIEGPPEGQHLRAGTRVRLVCLAIGGNPDPSLIWYKDSRTVTEPRSPQEPRRVQLGSLEKSGSTFSRELVLVTGPSDNRAKFTCKAGQLSASTQLVVQFPPTNVTILANASALRPGDALNLTCVSVSSNPPVSLSWDKEGERLESVAARPQSAPFKGSAAARTVLLRMSPRDHGHRVTCRAHSTKLQETVSAFYRLNVLYPPEFLGEQVLVVTAVEKGEALLPVSVSANPAPEAFNWTFRGYRLSPAGGPRHRILSGGALQLWNVTRADDGLYQLHCQNSEGTAEALVRLDVHYAPTIRALQDPTEVNIGGSVDIVCTVDANPILPEMFNWERLGEEVEDQSLDDMEKMSKGSTGRLRIHHAKLTQAGAYQCIVDNGVAPPARGLVRLVVRFAPHVEHPAPLTKVAAAGDSTSSATLHCRARGVPNIVFTWSKNGVPLDLQDPRYTEHTYHQGGIHSSLLTIANVSAAQDYALFTCTATNPLGSDHTNIQLVSISRPDPPSGLKVMSMTPNSVGLEWKPGFDGGLPQSFRIRYEALGTPGFLYMDVLPPQATTFTLTGLQPSTRYRVWLLASNALGDSGLADKGSQISITTPGLDQPSGEPNYQLPTEQPAGPSELP

SEQ ID NO: 12 - protein, 1065 aa, synthetic construct
  source 1..1065: note = pre-Nephrin(ec)[human]-His
MALGTTLRASLLLLGLLTEGLAQLAIPASVPRGFWALPENLTVVEGASVELRCGVSTPGSAVQWAKDGLLLGPDPRIPGFPRYRLEGDPARGEFHLHIEACDLSDDAEYECQVGRSEMGPELVSPRVILSILVPPKLLLLTPEAGTMVTWVAGQEYVVNCVSGDAKPAPDITILLSGQTISDISANVNEGSQQKLFTVEATARVTPRSSDNRQLLVCEASSPALEAPIKASFTVNVLFPPGPPVIEWPGLDEGHVRAGQSLELPCVARGGNPLATLQWLKNGQPVSTAWGTEHTQAVARSVLVMTVRPEDHGAQLSCEAHNSVSAGTQEHGITLQVTFPPSAIIILGSASQTENKNVTLSCVSKSSRPRVLLRWWLGWRQLLPMEETVMDGLHGGHISMSNLTFLARREDNGLTLTCEAFSEAFTKETFKKSLILNVKYPAQKLWIEGPPEGQKLRAGTRVRLVCLAIGGNPEPSLMWYKDSRTVTESRLPQESRRVHLGSVEKSGSTFSRELVLVTGPSDNQAKFTCKAGQLSASTQLAVQFPPTNVTILANASALRPGDALNLTCVSVSSNPPVNLSWDKEGERLEGVAAPPRRAPFKGSAAARSVLLQVSSRDHGQRVTCRAHSAELRETVSSFYRLNVLYRPEFLGEQVLVVTAVEQGEALLPVSVSANPAPEAFNWTFRGYRLSPAGGPRHRILSSGALHLWNVTRADDGLYQLHCQNSEGTAEARLRLDVHYAPTIRALQDPTEVNVGGSVDIVCTVDANPILPGMFNWERLGEDEEDQSLDDMEKISRGPTGRLRIHHAKLAQAGAYQCIVDNGVAPPARRLLRLVVRFAPQVEHPTPLTKVAAAGDSTSSATLHCRARGVPNIVFTWTKNGVPLDLQDPRYTEHTYHQGGVHSSLLTIANVSAAQDYALFTCTATNALGSDQTNIQLVSISRPDPPSGLKVVSLTPHSVGLEWKPGFDGGLPQRFCIRYEALGTPGFHYVDVVPPQATTFTLTGLQPSTRYRVWLLASNALGDSGLADKGTQLPITTPGLHQPSGEPEDQLPTEPPSLEHHHHHHHH

SEQ ID NO: 13 - protein, 1088 aa, synthetic construct
  source 1..1088: note = pre-Nephrin(ec)[human]-H8-avi-b
MALGTTLRASLLLLGLLTEGLAQLAIPASVPRGFWALPENLTVVEGASVELRCGVSTPGSAVQWAKDGLLLGPDPRIPGFPRYRLEGDPARGEFHLHIEACDLSDDAEYECQVGRSEMGPELVSPRVILSILVPPKLLLLTPEAGTMVTWVAGQEYVVNCVSGDAKPAPDITILLSGQTISDISANVNEGSQQKLFTVEATARVTPRSSDNRQLLVCEASSPALEAPIKASFTVNVLFPPGPPVIEWPGLDEGHVRAGQSLELPCVARGGNPLATLQWLKNGQPVSTAWGTEHTQAVARSVLVMTVRPEDHGAQLSCEAHNSVSAGTQEHGITLQVTFPPSAIIILGSASQTENKNVTLSCVSKSSRPRVLLRWWLGWRQLLPMEETVMDGLHGGHISMSNLTFLARREDNGLTLTCEAFSEAFTKETFKKSLILNVKYPAQKLWIEGPPEGQKLRAGTRVRLVCLAIGGNPEPSLMWYKDSRTVTESRLPQESRRVHLGSVEKSGSTFSRELVLVTGPSDNQAKFTCKAGQLSASTQLAVQFPPTNVTILANASALRPGDALNLTCVSVSSNPPVNLSWDKEGERLEGVAAPPRRAPFKGSAAARSVLLQVSSRDHGQRVTCRAHSAELRETVSSFYRLNVLYRPEFLGEQVLVVTAVEQGEALLPVSVSANPAPEAFNWTFRGYRLSPAGGPRHRILSSGALHLWNVTRADDGLYQLHCQNSEGTAEARLRLDVHYAPTIRALQDPTEVNVGGSVDIVCTVDANPILPGMFNWERLGEDEEDQSLDDMEKISRGPTGRLRIHHAKLAQAGAYQCIVDNGVAPPARRLLRLVVRFAPQVEHPTPLTKVAAAGDSTSSATLHCRARGVPNIVFTWTKNGVPLDLQDPRYTEHTYHQGGVHSSLLTIANVSAAQDYALFTCTATNALGSDQTNIQLVSISRPDPPSGLKVVSLTPHSVGLEWKPGFDGGLPQRFCIRYEALGTPGFHYVDVVPPQATTFTLTGLQPSTRYRVWLLASNALGDSGLADKGTQLPITTPGLHQPSGEPEDQLPTEPPSLEGSGSGSHHHHHHHHGSGLNDIFEAQKIEWHE

SEQ ID NO: 14 - protein, 1241 aa, Homo sapiens
  source 1..1241: note = pre-Nephrin[human]
MALGTTLRASLLLLGLLTEGLAQLAIPASVPRGFWALPENLTVVEGASVELRCGVSTPGSAVQWAKDGLLLGPDPRIPGFPRYRLEGDPARGEFHLHIEACDLSDDAEYECQVGRSEMGPELVSPRVILSILVPPKLLLLTPEAGTMVTWVAGQEYVVNCVSGDAKPAPDITILLSGQTISDISANVNEGSQQKLFTVEATARVTPRSSDNRQLLVCEASSPALEAPIKASFTVNVLFPPGPPVIEWPGLDEGHVRAGQSLELPCVARGGNPLATLQWLKNGQPVSTAWGTEHTQAVARSVLVMTVRPEDHGAQLSCEAHNSVSAGTQEHGITLQVTFPPSAIIILGSASQTENKNVTLSCVSKSSRPRVLLRWWLGWRQLLPMEETVMDGLHGGHISMSNLTFLARREDNGLTLTCEAFSEAFTKETFKKSLILNVKYPAQKLWIEGPPEGQKLRAGTRVRLVCLAIGGNPEPSLMWYKDSRTVTESRLPQESRRVHLGSVEKSGSTFSRELVLVTGPSDNQAKFTCKAGQLSASTQLAVQFPPTNVTILANASALRPGDALNLTCVSVSSNPPVNLSWDKEGERLEGVAAPPRRAPFKGSAAARSVLLQVSSRDHGQRVTCRAHSAELRETVSSFYRLNVLYRPEFLGEQVLVVTAVEQGEALLPVSVSANPAPEAFNWTFRGYRLSPAGGPRHRILSSGALHLWNVTRADDGLYQLHCQNSEGTAEARLRLDVHYAPTIRALQDPTEVNVGGSVDIVCTVDANPILPGMFNWERLGEDEEDQSLDDMEKISRGPTGRLRIHHAKLAQAGAYQCIVDNGVAPPARRLLRLVVRFAPQVEHPTPLTKVAAAGDSTSSATLHCRARGVPNIVFTWTKNGVPLDLQDPRYTEHTYHQGGVHSSLLTIANVSAAQDYALFTCTATNALGSDQTNIQLVSISRPDPPSGLKVVSLTPHSVGLEWKPGFDGGLPQRFCIRYEALGTPGFHYVDVVPPQATTFTLTGLQPSTRYRVWLLASNALGDSGLADKGTQLPITTPGLHQPSGEPEDQLPTEPPSGPSGLPLLPVLFALGGLLLLSNASCVGGVLWQRRLRRLAEGISEKTEAGSEEDRVRNEYEESQWTGERDTQSSTVSTTEAEPYYRSLRDFSPQLPPTQEEVSYSRGFTGEDEDMAFPGHLYDEVERTYPPSGAWGPLYDEVQMGPWDLHWPEDTYQDPRGIYDQVAGDLDTLEPDSLPFELRGHLV

SEQ ID NO: 15 - protein, 353 aa, Homo sapiens
ASPTSPKVFPLSLCSTQPDGNVVIACLVQGFFPQEPLSVTWSESGQGVTARNFPPSQDASGDLYTTSSQLTLPATQCLAGKSVTCHVKHYTNPSQDVTVPCPVPSTPPTPSPSTPPTPSPSCCHPRLSLHRPALEDLLLGSEANLTCTLTGLRDASGVTFTWTPSSGKSAVQGPPERDLCGCYSVSSVLPGCAEPWNHGKTFTCTAAYPESKTPLTATLSKSGNTFRPEVHLLPPPSEELALNELVTLTCLARGFSPKDVLVRWLQGSQELPREKYLTWASRQEPSQGTTTFAVTSILRVAAEDWKKGDTFSCMVGHEALPLAFTQKTIDRLAGKPTHVNVSVVMAEVDGTCY

SEQ ID NO: 16 - protein, 340 aa, Homo sapiens
ASPTSPKVFPLSLDSTPQDGNVVVACLVQGFFPQEPLSVTWSESGQNVTARNFPPSQDASGDLYTTSSQLTLPATQCPDGKSVTCHVKHYTNSSQDVTVPCRVPPPPPCCHPRLSLHRPALEDLLLGSEANLTCTLTGLRDASGATFTWTPSSGKSAVQGPPERDLCGCYSVSSVLPGCAQPWNHGETFTCTAAHPELKTPLTANITKSGNTFRPEVHLLPPPSEELALNELVTLTCLARGFSPKDVLVRWLQGSQELPREKYLTWASRQEPSQGTTTYAVTSILRVAAEDWKKGETFSCMVGHEALPLAFTQKTIDRMAGKPTHINVSVVMAEADGTCY

SEQ ID NO: 17 - protein, 384 aa, Homo sapiens
APTKAPDVFPIISGCRHPKDNSPVVLACLITGYHPTSVTVTWYMGTQSQPQRTFPEIQRRDSYYMTSSQLSTPLQQWRQGEYKCVVQHTASKSKKEIFRWPESPKAQASSVPTAQPQAEGSLAKATTAPATTRNTGRGGEEKKKEKEKEEQEERETKTPECPSHTQPLGVYLLTPAVQDLWLRDKATFTCFVVGSDLKDAHLTWEVAGKVPTGGVEEGLLERHSNGSQSQHSRLTLPRSLWNAGTSVTCTLNHPSLPPQRLMALREPAAQAPVKLSLNLLASSDPPEAASWLLCEVSGFSPPNILLMWLEDQREVNTSGFAPARPPPQPRSTTFWAWSVLRVPAPPSPQPATYTCVVSHEDSRTLLNASRSLEVSYVTDHGPMK

SEQ ID NO: 18 - protein, 428 aa, Homo sapiens
ASTQSPSVFPLTRCCKNIPSNATSVTLGCLATGYFPEPVMVTWDTGSLNGTTMTLPATTLTLSGHYATISLLTVSGAWAKQMFTCRVAHTPSSTDWVDNKTFSVCSRDFTPPTVKILQSSCDGGGHFPPTIQLLCLVSGYTPGTINITWLEDGQVMDVDLSTASTTQEGELASTQSELTLSQKHWLSDRTYTCQVTYQGHTFEDSTKKCADSNPRGVSAYLSRPSPFDLFIRKSPTITCLVVDLAPSKGTVNLTWSRASGKPVNHSTRKEEKQRNGTLTVTSTLPVGTRDWIEGETYQCRVTHPHLPRALMRSTTKTSGPRAAPEVYAFATPEWPGSRDKRTLACLIQNFMPEDISVQWLHNEVQLPDARHSTTQPRKTKGSGFFVFSRLEVTRAEWEQKDEFICRAVHEAASPSQTVQRAVSVNPGK

SEQ ID NO: 19 - protein, 330 aa, Homo sapiens [sequence omitted]

SEQ ID NO: 20 - protein, 326 aa, Homo sapiens
ASTKGPSVFPLAPCSRSTSESTAALGCLVKDYFPEPVTVSWNSGALTSGVHTFPAVLQSSGLYSLSSVVTVPSSNFGTQTYTCNVDHKPSNTKVDKTVERKCCVECPPCPAPPVAGPSVFLFPPKPKDTLMISRTPEVTCVVVDVSHEDPEVQFNWYVDGVEVHNAKTKPREEQFNSTFRVVSVLTVVHQDWLNGKEYKCKVSNKGLPAPIEKTISKTKGQPREPQVYTLPPSREEMTKNQVSLTCLVKGFYPSDISVEWESNGQPENNYKTTPPMLDSDGSFFLYSKLTVDKSRWQQGNVFSCSVMHEALHNHYTQKSLSLSPGK

SEQ ID NO: 21 - protein, 377 aa, Homo sapiens
ASTKGPSVFPLAPCSRSTSGGTAALGCLVKDYFPEPVTVSWNSGALTSGVHTFPAVLQSSGLYSLSSVVTVPSSSLGTQTYTCNVNHKPSNTKVDKRVELKTPLGDTTHTCPRCPEPKSCDTPPPCPRCPEPKSCDTPPPCPRCPEPKSCDTPPPCPRCPAPELLGGPSVFLFPPKPKDTLMISRTPEVTCVVVDVSHEDPEVQFKWYVDGVEVHNAKTKPREEQYNSTFRVVSVLTVLHQDWLNGKEYKCKVSNKALPAPIEKTISKTKGQPREPQVYTLPPSREEMTKNQVSLTCLVKGFYPSDIAVEWESSGQPENNYNTTPPMLDSDGSFFLYSKLTVDKSRWQQGNIFSCSVMHEALHNRFTQKSLSLSPGK

SEQ ID NO: 22 - protein, 327 aa, Homo sapiens
ASTKGPSVFPLAPCSRSTSESTAALGCLVKDYFPEPVTVSWNSGALTSGVHTFPAVLQSSGLYSLSSVVTVPSSSLGTKTYTCNVDHKPSNTKVDKRVESKYGPPCPSCPAPEFLGGPSVFLFPPKPKDTLMISRTPEVTCVVVDVSQEDPEVQFNWYVDGVEVHNAKTKPREEQFNSTYRVVSVLTVLHQDWLNGKEYKCKVSNKGLPSSIEKTISKAKGQPREPQVYTLPPSQEEMTKNQVSLTCLVKGFYPSDIAVEWESNGQPENNYKTTPPVLDSDGSFFLYSRLTVDKSRWQEGNVFSCSVMHEALHNHYTQKSLSLSLGK

SEQ ID NO: 23 - protein, 453 aa, Homo sapiens
GSASAPTLFPLVSCENSPSDTSSVAVGCLAQDFLPDSITFSWKYKNNSDISSTRGFPSVLRGGKYAATSQVLLPSKDVMQGTDEHVVCKVQHPNGNKEKNVPLPVIAELPPKVSVFVPPRDGFFGNPRKSKLICQATGFSPRQIQVSWLREGKQVGSGVTTDQVQAEAKESGPTTYKVTSTLTIKESDWLGQSMFTCRVDHRGLTFQQNASSMCVPDQDTAIRVFAIPPSFASIFLTKSTKLTCLVTDLTTYDSVTISWTRQNGEAVKTHTNISESHPNATFSAVGEASICEDDWNSGERFTCTVTHTDLPSPLKQTISRPKGVALHRPDVYLLPPAREQLNLRESATITCLVTGFSPADVFVQWMQRGQPLSPEKYVTSAPMPEPQAPGRYFAHSILTVSEEEWNTGETYTCVVAHEALPNRVTERTVDKSTGKPTLYNVSLVMSDTAGTCY

SEQ ID NO: 24 - protein, 106 aa, Homo sapiens
GQPKANPTVTLFPPSSEELQANKATLVCLISDFYPGAVTVAWKADGSPVKAGVETTKPSKQSNNKYAASSYLSLTPEQWKSHRSYSCQVTHEGSTVEKTVAPTECS

SEQ ID NO: 25 - protein, 106 aa, Homo sapiens
GQPKAAPSVTLFPPSSEELQANKATLVCLISDFYPGAVTVAWKADSSPVKAGVETTTPSKQSNNKYAASSYLSLTPEQWKSHRSYSCQVTHEGSTVEKTVAPTECS

SEQ ID NO: 26 - protein, 106 aa, Homo sapiens
GQPKAAPSVTLFPPSSEELQANKATLVCLISDFYPGAVTVAWKADSSPVKAGVETTTPSKQSNNKYAASSYLSLTPEQWKSHKSYSCQVTHEGSTVEKTVAPTECS

SEQ ID NO: 27 - protein, 106 aa, Homo sapiens
GQPKAAPSVTLFPPSSEELQANKATLVCLISDFYPGAVKVAWKADGSPVNTGVETTTPSKQSNNKYAASSYLSLTPEQWKSHRSYSCQVTHEGSTVEKTVAPAECS

SEQ ID NO: 28 - protein, 106 aa, Homo sapiens
GQPKAAPSVTLFPPSSEELQANKATLVCLVSDFNPGAVTVAWKADGSPVKVGVETTKPSKQSNNKYAASSYLSLTPEQWKSHRSYSCRVTHEGSTVEKTVAPAECS

SEQ ID NO: 29 - protein, 107 aa, Homo sapiens [sequence omitted]

SEQ ID NO: 30 - protein, 12 aa, synthetic construct
VGRSEMGPELVS

SEQ ID NO: 31 - protein, 11 aa, synthetic construct
PPKLLLLTPEA

SEQ ID NO: 32 - protein, 11 aa, synthetic construct
LSGQTISDISA

SEQ ID NO: 33 - protein, 12 aa, synthetic construct
NGQPVSTAWGTE

SEQ ID NO: 34 - protein, 19 aa, synthetic construct
HNSVSAGTQEHGITLQVTF

SEQ ID NO: 35 - protein, 17 aa, synthetic construct
SGQTISDISANVNGSQQ

SEQ ID NO: 36 - protein, 13 aa, synthetic construct
QLSCEAHNSVSAG

SEQ ID NO: 37 - protein, 20 aa, synthetic construct
SPALEAPIKASFTVNVLFPP

SEQ ID NO: 38 - protein, 14 aa, synthetic construct
IEWPGLDEGHVRAG

SEQ ID NO: 39 - protein, 13 aa, synthetic construct
PPEGQKLRAGTRV

SEQ ID NO: 40 - protein, 12 aa, synthetic construct
PEPSLMWYKDSR

SEQ ID NO: 41 - protein, 12 aa, synthetic construct
RYEALGTPGFHY

SEQ ID NO: 42 - protein, 11 aa, synthetic construct
VDVVPPQATTF

SEQ ID NO: 43 - protein, 45 aa, synthetic construct
VGRSEMGPELVSLEGSGSGSHHHHHHHHGSGLNDIFEAQKIEWHE

SEQ ID NO: 44 - protein, 44 aa, synthetic construct
PPKLLLLTPEALEGSGSGSHHHHHHHHGSGLNDIFEAQKIEWHE

SEQ ID NO: 45 - protein, 44 aa, synthetic construct
LSGQTISDISALEGSGSGSHHHHHHHHGSGLNDIFEAQKIEWHE

SEQ ID NO: 46 - protein, 45 aa, synthetic construct
NGQPVSTAWGTELEGSGSGSHHHHHHHHGSGLNDIFEAQKIEWHE

SEQ ID NO: 47 - protein, 52 aa, synthetic construct
HNSVSAGTQEHGITLQVTFLEGSGSGSHHHHHHHHGSGLNDIFEAQKIEWHE

SEQ ID NO: 48 - protein, 50 aa, synthetic construct
SGQTISDISANVNGSQQLEGSGSGSHHHHHHHHGSGLNDIFEAQKIEWHE

SEQ ID NO: 49 - protein, 46 aa, synthetic construct
QLSCEAHNSVSAGLEGSGSGSHHHHHHHHGSGLNDIFEAQKIEWHE

SEQ ID NO: 50 - protein, 53 aa, synthetic construct
SPALEAPIKASFTVNVLFPPLEGSGSGSHHHHHHHHGSGLNDIFEAQKIEWHE

SEQ ID NO: 51 - protein, 47 aa, synthetic construct
IEWPGLDEGHVRAGLEGSGSGSHHHHHHHHGSGLNDIFEAQKIEWHE

SEQ ID NO: 52 - protein, 46 aa, synthetic construct
PPEGQKLRAGTRVLEGSGSGSHHHHHHHHGSGLNDIFEAQKIEWHE

SEQ ID NO: 53 - protein, 45 aa, synthetic construct
PEPSLMWYKDSRLEGSGSGSHHHHHHHHGSGLNDIFEAQKIEWHE

SEQ ID NO: 54 - protein, 45 aa, synthetic construct
RYEALGTPGFHYLEGSGSGSHHHHHHHHGSGLNDIFEAQKIEWHE

SEQ ID NO: 55 - protein, 44 aa, synthetic construct
VDVVPPQATTFLEGSGSGSHHHHHHHHGSGLNDIFEAQKIEWHE

SEQ ID NO: 56 - protein, 45 aa, synthetic construct
VGRSEAGPELVSLEGSGSGSHHHHHHHHGSGLNDIFEAQKIEWHE

SEQ ID NO: 57 - protein, 45 aa, synthetic construct
VGRSETGPELVSLEGSGSGSHHHHHHHHGSGLNDIFEAQKIEWHE

SEQ ID NO: 58 - protein, 44 aa, synthetic construct
PPKLLALTPEALEGSGSGSHHHHHHHHGSGLNDIFEAQKIEWHE

SEQ ID NO: 59 - protein, 44 aa, synthetic construct
PPKLLQLTPEALEGSGSGSHHHHHHHHGSGLNDIFEAQKIEWHE

SEQ ID NO: 60 - protein, 44 aa, synthetic construct
LSGQTASDISALEGSGSGSHHHHHHHHGSGLNDIFEAQKIEWHE

SEQ ID NO: 61 - protein, 44 aa, synthetic construct
LSGQTVSDISALEGSGSGSHHHHHHHHGSGLNDIFEAQKIEWHE

SEQ ID NO: 62 - protein, 45 aa, synthetic construct
NGQPVSAAWGTELEGSGSGSHHHHHHHHGSGLNDIFEAQKIEWHE

SEQ ID NO: 63 - protein, 45 aa, synthetic construct
NGQPVSIAWGTELEGSGSGSHHHHHHHHGSGLNDIFEAQKIEWHE

SEQ ID NO: 64 - protein, 52 aa, synthetic construct
HNSVSAATQEAAITLQVTFLEGSGSGSHHHHHHHHGSGLNDIFEAQKIEWHE

SEQ ID NO: 65 - protein, 52 aa, synthetic construct
HNSVSAETQERSITLQVTFLEGSGSGSHHHHHHHHGSGLNDIFEAQKIEWHE

SEQ ID NO: 66 - protein, 50 aa, synthetic construct
SGQTIADASANVNGSQQLEGSGSGSHHHHHHHHGSGLNDIFEAQKIEWHE

SEQ ID NO: 67 - protein, 50 aa, synthetic construct
SGQTILDVSSNVNGSQQLEGSGSGSHHHHHHHHGSGLNDIFEAQKIEWHE

SEQ ID NO: 68 - protein, 46 aa, synthetic construct
QLSCEAANSVSAGLEGSGSGSHHHHHHHHGSGLNDIFEAQKIEWHE

SEQ ID NO: 69 - protein, 46 aa, synthetic construct
QLSCEAYNSVSAGLEGSGSGSHHHHHHHHGSGLNDIFEAQKIEWHE

SEQ ID NO: 70 - protein, 53 aa, synthetic construct
SPALAAPIKASATANVLFPPLEGSGSGSHHHHHHHHGSGLNDIFEAQKIEWHE

SEQ ID NO: 71 - protein, 53 aa, synthetic construct
SPALVSPIKVSITMNVLFPPLEGSGSGSHHHHHHHHGSGLNDIFEAQKIEWHE

SEQ ID NO: 72 - protein, 47 aa, synthetic construct
IEWPGLAEGHVRAGLEGSGSGSHHHHHHHHGSGLNDIFEAQKIEWHE

SEQ ID NO: 73 - protein, 47 aa, synthetic construct
IEWPGLNEGHVRAGLEGSGSGSHHHHHHHHGSGLNDIFEAQKIEWHE

SEQ ID NO: 74 - protein, 46 aa, synthetic construct
PPEGQALRAGTRVLEGSGSGSHHHHHHHHGSGLNDIFEAQKIEWHE

SEQ ID NO: 75 - protein, 46 aa, synthetic construct
PPEGQRLRAGTRVLEGSGSGSHHHHHHHHGSGLNDIFEAQKIEWHE

SEQ ID NO: 76 - protein, 45 aa, synthetic construct
PEPSLAWYKDSRLEGSGSGSHHHHHHHHGSGLNDIFEAQKIEWHE

SEQ ID NO: 77 - protein, 45 aa, synthetic construct
PEPSLTWYKDSRLEGSGSGSHHHHHHHHGSGLNDIFEAQKIEWHE

SEQ ID NO: 78 - protein, 45 aa, synthetic construct
RYEALATPGFHYLEGSGSGSHHHHHHHHGSGLNDIFEAQKIEWHE

SEQ ID NO: 79 - protein, 45 aa, synthetic construct
RYEALDTPGFHYLEGSGSGSHHHHHHHHGSGLNDIFEAQKIEWHE

SEQ ID NO: 80 - protein, 44 aa, synthetic construct
VDVVPAQATTFLEGSGSGSHHHHHHHHGSGLNDIFEAQKIEWHE

SEQ ID NO: 81 - protein, 1070 aa, synthetic construct
MALGTTLRASLLLLGLLTEGLAQLAIPASVPRGFWALPENLTVVEGASVELRCGVSTPGSAVQWAKDGLLLGPDPRIPGFPRYRLEGDPARGEFHLHIEACDLSDDAEYECQVGRSEMGPELVSPRVILSILVPPKLLLLTPEAGTMVTWVAGQEYVVNCVSGDAKPAPDITILLSGQTISDISANVNEGSQQKLFTVEATARVTPRSSDNRQLLVCEASSPALEAPIKASFTVNVLFPPGPPVIEWPGLDEGHVRAGQSLELPCVARGGNPLATLQWLKNGQPVSAAWGTEHTQAVARSVLVMTVRPEDHGAQLSCEAHNSVSAGTQEHGITLQVTFPPSAIIILGSASQTENKNVTLSCVSKSSRPRVLLRWWLGWRQLLPMEETVMDGLHGGHISMSNLTFLARREDNGLTLTCEAFSEAFTKETFKKSLILNVKYPAQKLWIEGPPEGQKLRAGTRVRLVCLAIGGNPEPSLMWYKDSRTVTESRLPQESRRVHLGSVEKSGSTFSRELVLVTGPSDNQAKFTCKAGQLSASTQLAVQFPPTNVTILANASALRPGDALNLTCVSVSSNPPVNLSWDKEGERLEGVAAPPRRAPFKGSAAARSVLLQVSSRDHGQRVTCRAHSAELRETVSSFYRLNVLYRPEFLGEQVLVVTAVEQGEALLPVSVSANPAPEAFNWTFRGYRLSPAGGPRHRILSSGALHLWNVTRADDGLYQLHCQNSEGTAEARLRLDVHYAPTIRALQDPTEVNVGGSVDIVCTVDANPILPGMFNWERLGEDEEDQSLDDMEKISRGPTGRLRIHHAKLAQAGAYQCIVDNGVAPPARRLLRLVVRFAPQVEHPTPLTKVAAAGDSTSSATLHCRARGVPNIVFTWTKNGVPLDLQDPRYTEHTYHQGGVHSSLLTIANVSAAQDYALFTCTATNALGSDQTNIQLVSISRPDPPSGLKVVSLTPHSVGLEWKPGFDGGLPQRFCIRYEALGTPGFHYVDVVPPQATTFTLTGLQPSTRYRVWLLASNALGDSGLADKGTQLPITTPGLEGSGSGSHHHHHHHHGSGLNDIFEAQKIEWHE

SEQ ID NO: 82 - protein, 1070 aa, synthetic construct
MALGTTLRASLLLLGLLTEGLAQLAIPASVPRGFWALPENLTVVEGASVELRCGVSTPGSAVQWAKDGLLLGPDPRIPGFPRYRLEGDPARGEFHLHIEACDLSDDAEYECQVGRSEMGPELVSPRVILSILVPPKLLLLTPEAGTMVTWVAGQEYVVNCVSGDAKPAPDITILLSGQTISDISANVNEGSQQKLFTVEATARVTPRSSDNRQLLVCEASSPALEAPIKASFTVNVLFPPGPPVIEWPGLDEGHVRAGQSLELPCVARGGNPLATLQWLKNGQPVSIAWGTEHTQAVARSVLVMTVRPEDHGAQLSCEAHNSVSAGTQEHGITLQVTFPPSAIIILGSASQTENKNVTLSCVSKSSRPRVLLRWWLGWRQLLPMEETVMDGLHGGHISMSNLTFLARREDNGLTLTCEAFSEAFTKETFKKSLILNVKYPAQKLWIEGPPEGQKLRAGTRVRLVCLAIGGNPEPSLMWYKDSRTVTESRLPQESRRVHLGSVEKSGSTFSRELVLVTGPSDNQAKFTCKAGQLSASTQLAVQFPPTNVTILANASALRPGDALNLTCVSVSSNPPVNLSWDKEGERLEGVAAPPRRAPFKGSAAARSVLLQVSSRDHGQRVTCRAHSAELRETVSSFYRLNVLYRPEFLGEQVLVVTAVEQGEALLPVSVSANPAPEAFNWTFRGYRLSPAGGPRHRILSSGALHLWNVTRADDGLYQLHCQNSEGTAEARLRLDVHYAPTIRALQDPTEVNVGGSVDIVCTVDANPILPGMFNWERLGEDEEDQSLDDMEKISRGPTGRLRIHHAKLAQAGAYQCIVDNGVAPPARRLLRLVVRFAPQVEHPTPLTKVAAAGDSTSSATLHCRARGVPNIVFTWTKNGVPLDLQDPRYTEHTYHQGGVHSSLLTIANVSAAQDYALFTCTATNALGSDQTNIQLVSISRPDPPSGLKVVSLTPHSVGLEWKPGFDGGLPQRFCIRYEALGTPGFHYVDVVPPQATTFTLTGLQPSTRYRVWLLASNALGDSGLADKGTQLPITTPGLEGSGSGSHHHHHHHHGSGLNDIFEAQKIEWHE

SEQ ID NO: 83 - protein, 1070 aa, synthetic construct
MALGTTLRASLLLLGLLTEGLAQLAIPASVPRGFWALPENLTVVEGASVELRCGVSTPGSAVQWAKDGLLLGPDPRIPGFPRYRLEGDPARGEFHLHIEACDLSDDAEYECQVGRSEMGPELVSPRVILSILVPPKLLLLTPEAGTMVTWVAGQEYVVNCVSGDAKPAPDITILLSGQTISDISANVNEGSQQKLFTVEATARVTPRSSDNRQLLVCEASSPALEAPIKASFTVNVLFPPGPPVIEWPGLDEGHVRAGQSLELPCVARGGNPLATLQWLKNGQPVSTAWGTEHTQAVARSVLVMTVRPEDHGAQLSCEAHNSVSAATQEAAITLQVTFPPSAIIILGSASQTENKNVTLSCVSKSSRPRVLLRWWLGWRQLLPMEETVMDGLHGGHISMSNLTFLARREDNGLTLTCEAFSEAFTKETFKKSLILNVKYPAQKLWIEGPPEGQKLRAGTRVRLVCLAIGGNPEPSLMWYKDSRTVTESRLPQESRRVHLGSVEKSGSTFSRELVLVTGPSDNQAKFTCKAGQLSASTQLAVQFPPTNVTILANASALRPGDALNLTCVSVSSNPPVNLSWDKEGERLEGVAAPPRRAPFKGSAAARSVLLQVSSRDHGQRVTCRAHSAELRETVSSFYRLNVLYRPEFLGEQVLVVTAVEQGEALLPVSVSANPAPEAFNWTFRGYRLSPAGGPRHRILSSGALHLWNVTRADDGLYQLHCQNSEGTAEARLRLDVHYAPTIRALQDPTEVNVGGSVDIVCTVDANPILPGMFNWERLGEDEEDQSLDDMEKISRGPTGRLRIHHAKLAQAGAYQCIVDNGVAPPARRLLRLVVRFAPQVEHPTPLTKVAAAGDSTSSATLHCRARGVPNIVFTWTKNGVPLDLQDPRYTEHTYHQGGVHSSLLTIANVSAAQDYALFTCTATNALGSDQTNIQLVSISRPDPPSGLKVVSLTPHSVGLEWKPGFDGGLPQRFCIRYEALGTPGFHYVDVVPPQATTFTLTGLQPSTRYRVWLLASNALGDSGLADKGTQLPITTPGLEGSGSGSHHHHHHHHGSGLNDIFEAQKIEWHE

SEQ ID NO: 84 - protein, 1070 aa, synthetic construct
MALGTTLRASLLLLGLLTEGLAQLAIPASVPRGFWALPENLTVVEGASVELRCGVSTPGSAVQWAKDGLLLGPDPRIPGFPRYRLEGDPARGEFHLHIEACDLSDDAEYECQVGRSEMGPELVSPRVILSILVPPKLLLLTPEAGTMVTWVAGQEYVVNCVSGDAKPAPDITILLSGQTISDISANVNEGSQQKLFTVEATARVTPRSSDNRQLLVCEASSPALEAPIKASFTVNVLFPPGPPVIEWPGLDEGHVRAGQSLELPCVARGGNPLATLQWLKNGQPVSTAWGTEHTQAVARSVLVMTVRPEDHGAQLSCEAHNSVSAETQERSITLQVTFPPSAIIILGSASQTENKNVTLSCVSKSSRPRVLLRWWLGWRQLLPMEETVMDGLHGGHISMSNLTFLARREDNGLTLTCEAFSEAFTKETFKKSLILNVKYPAQKLWIEGPPEGQKLRAGTRVRLVCLAIGGNPEPSLMWYKDSRTVTESRLPQESRRVHLGSVEKSGSTFSRELVLVTGPSDNQAKFTCKAGQLSASTQLAVQFPPTNVTILANASALRPGDALNLTCVSVSSNPPVNLSWDKEGERLEGVAAPPRRAPFKGSAAARSVLLQVSSRDHGQRVTCRAHSAELRETVSSFYRLNVLYRPEFLGEQVLVVTAVEQGEALLPVSVSANPAPEAFNWTFRGYRLSPAGGPRHRILSSGALHLWNVTRADDGLYQLHCQNSEGTAEARLRLDVHYAPTIRALQDPTEVNVGGSVDIVCTVDANPILPGMFNWERLGEDEEDQSLDDMEKISRGPTGRLRIHHAKLAQAGAYQCIVDNGVAPPARRLLRLVVRFAPQVEHPTPLTKVAAAGDSTSSATLHCRARGVPNIVFTWTKNGVPLDLQDPRYTEHTYHQGGVHSSLLTIANVSAAQDYALFTCTATNALGSDQTNIQLVSISRPDPPSGLKVVSLTPHSVGLEWKPGFDGGLPQRFCIRYEALGTPGFHYVDVVPPQATTFTLTGLQPSTRYRVWLLASNALGDSGLADKGTQLPITTPGLEGSGSGSHHHHHHHHGSGLNDIFEAQKIEWHE

SEQ ID NO: 85 - protein, 1070 aa, synthetic construct
MALGTTLRASLLLLGLLTEGLAQLAIPASVPRGFWALPENLTVVEGASVELRCGVSTPGSAVQWAKDGLLLGPDPRIPGFPRYRLEGDPARGEFHLHIEACDLSDDAEYECQVGRSEMGPELVSPRVILSILVPPKLLLLTPEAGTMVTWVAGQEYVVNCVSGDAKPAPDITILLSGQTIADASANVNEGSQQKLFTVEATARVTPRSSDNRQLLVCEASSPALEAPIKASFTVNVLFPPGPPVIEWPGLDEGHVRAGQSLELPCVARGGNPLATLQWLKNGQPVSTAWGTEHTQAVARSVLVMTVRPEDHGAQLSCEAHNSVSAGTQEHGITLQVTFPPSAIIILGSASQTENKNVTLSCVSKSSRPRVLLRWWLGWRQLLPMEETVMDGLHGGHISMSNLTFLARREDNGLTLTCEAFSEAFTKETFKKSLILNVKYPAQKLWIEGPPEGQKLRAGTRVRLVCLAIGGNPEPSLMWYKDSRTVTESRLPQESRRVHLGSVEKSGSTFSRELVLVTGPSDNQAKFTCKAGQLSASTQLAVQFPPTNVTILANASALRPGDALNLTCVSVSSNPPVNLSWDKEGERLEGVAAPPRRAPFKGSAAARSVLLQVSSRDHGQRVTCRAHSAELRETVSSFYRLNVLYRPEFLGEQVLVVTAVEQGEALLPVSVSANPAPEAFNWTFRGYRLSPAGGPRHRILSSGALHLWNVTRADDGLYQLHCQNSEGTAEARLRLDVHYAPTIRALQDPTEVNVGGSVDIVCTVDANPILPGMFNWERLGEDEEDQSLDDMEKISRGPTGRLRIHHAKLAQAGAYQCIVDNGVAPPARRLLRLVVRFAPQVEHPTPLTKVAAAGDSTSSATLHCRARGVPNIVFTWTKNGVPLDLQDPRYTEHTYHQGGVHSSLLTIANVSAAQDYALFTCTATNALGSDQTNIQLVSISRPDPPSGLKVVSLTPHSVGLEWKPGFDGGLPQRFCIRYEALGTPGFHYVDVVPPQATTFTLTGLQPSTRYRVWLLASNALGDSGLADKGTQLPITTPGLEGSGSGSHHHHHHHHGSGLNDIFEAQKIEWHE

SEQ ID NO: 86 - protein, 1070 aa, synthetic construct; identical to SEQ ID NO: 85

SEQ ID NO: 87 - protein, 1070 aa, synthetic construct
MALGTTLRASLLLLGLLTEGLAQLAIPASVPRGFWALPENLTVVEGASVELRCGVSTPGSAVQWAKDGLLLGPDPRIPGFPRYRLEGDPARGEFHLHIEACDLSDDAEYECQVGRSEMGPELVSPRVILSILVPPKLLLLTPEAGTMVTWVAGQEYVVNCVSGDAKPAPDITILLSGQTILDVSSNVNEGSQQKLFTVEATARVTPRSSDNRQLLVCEASSPALEAPIKASFTVNVLFPPGPPVIEWPGLDEGHVRAGQSLELPCVARGGNPLATLQWLKNGQPVSTAWGTEHTQAVARSVLVMTVRPEDHGAQLSCEAHNSVSAGTQEHGITLQVTFPPSAIIILGSASQTENKNVTLSCVSKSSRPRVLLRWWLGWRQLLPMEETVMDGLHGGHISMSNLTFLARREDNGLTLTCEAFSEAFTKETFKKSLILNVKYPAQKLWIEGPPEGQKLRAGTRVRLVCLAIGGNPEPSLMWYKDSRTVTESRLPQESRRVHLGSVEKSGSTFSRELVLVTGPSDNQAKFTCKAGQLSASTQLAVQFPPTNVTILANASALRPGDALNLTCVSVSSNPPVNLSWDKEGERLEGVAAPPRRAPFKGSAAARSVLLQVSSRDHGQRVTCRAHSAELRETVSSFYRLNVLYRPEFLGEQVLVVTAVEQGEALLPVSVSANPAPEAFNWTFRGYRLSPAGGPRHRILSSGALHLWNVTRADDGLYQLHCQNSEGTAEARLRLDVHYAPTIRALQDPTEVNVGGSVDIVCTVDANPILPGMFNWERLGEDEEDQSLDDMEKISRGPTGRLRIHHAKLAQAGAYQCIVDNGVAPPARRLLRLVVRFAPQVEHPTPLTKVAAAGDSTSSATLHCRARGVPNIVFTWTKNGVPLDLQDPRYTEHTYHQGGVHSSLLTIANVSAAQDYALFTCTATNALGSDQTNIQLVSISRPDPPSGLKVVSLTPHSVGLEWKPGFDGGLPQRFCIRYEALGTPGFHYVDVVPPQATTFTLTGLQPSTRYRVWLLASNALGDSGLADKGTQLPITTPGLEGSGSGSHHHHHHHHGSGLNDIFEAQKIEWHE

SEQ ID NO: 88 - protein, 1070 aa, synthetic construct
MALGTTLRASLLLLGLLTEGLAQLAIPASVPRGFWALPENLTVVEGASVELRCGVSTPGSAVQWAKDGLLLGPDPRIPGFPRYRLEGDPARGEFHLHIEACDLSDDAEYECQVGRSEMGPELVSPRVILSILVPPKLLLLTPEAGTMVTWVAGQEYVVNCVSGDAKPAPDITILLSGQTISDISANVNEGSQQKLFTVEATARVTPRSSDNRQLLVCEASSPALEAPIKASFTVNVLFPPGPPVIEWPGLDEGHVRAGQSLELPCVARGGNPLATLQWLKNGQPVSTAWGTEHTQAVARSVLVMTVRPEDHGAQLSCEAANSVSAGTQEHGITLQVTFPPSAIIILGSASQTENKNVTLSCVSKSSRPRVLLRWWLGWRQLLPMEETVMDGLHGGHISMSNLTFLARREDNGLTLTCEAFSEAFTKETFKKSLILNVKYPAQKLWIEGPPEGQKLRAGTRVRLVCLAIGGNPEPSLMWYKDSRTVTESRLPQESRRVHLGSVEKSGSTFSRELVLVTGPSDNQAKFTCKAGQLSASTQLAVQFPPTNVTILANASALRPGDALNLTCVSVSSNPPVNLSWDKEGERLEGVAAPPRRAPFKGSAAARSVLLQVSSRDHGQRVTCRAHSAELRETVSSFYRLNVLYRPEFLGEQVLVVTAVEQGEALLPVSVSANPAPEAFNWTFRGYRLSPAGGPRHRILSSGALHLWNVTRADDGLYQLHCQNSEGTAEARLRLDVHYAPTIRALQDPTEVNVGGSVDIVCTVDANPILPGMFNWERLGEDEEDQSLDDMEKISRGPTGRLRIHHAKLAQAGAYQCIVDNGVAPPARRLLRLVVRFAPQVEHPTPLTKVAAAGDSTSSATLHCRARGVPNIVFTWTKNGVPLDLQDPRYTEHTYHQGGVHSSLLTIANVSAAQDYALFTCTATNALGSDQTNIQLVSISRPDPPSGLKVVSLTPHSVGLEWKPGFDGGLPQRFCIRYEALGTPGFHYVDVVPPQATTFTLTGLQPSTRYRVWLLASNALGDSGLADKGTQLPITTPGLEGSGSGSHHHHHHHHGSGLNDIFEAQKIEWHE

SEQ ID NO: 89 - protein, 1070 aa, synthetic construct
MALGTTLRASLLLLGLLTEGLAQLAIPASVPRGFWALPENLTVVEGASVELRCGVSTPGSAVQWAKDGLLLGPDPRIPGFPRYRLEGDPARGEFHLHIEACDLSDDAEYECQVGRSEMGPELVSPRVILSILVPPKLLLLTPEAGTMVTWVAGQEYVVNCVSGDAKPAPDITILLSGQTISDISANVNEGSQQKLFTVEATARVTPRSSDNRQLLVCEASSPALEAPIKASFTVNVLFPPGPPVIEWPGLDEGHVRAGQSLELPCVARGGNPLATLQWLKNGQPVSTAWGTEHTQAVARSVLVMTVRPEDHGAQLSCEAYNSVSAGTQEHGITLQVTFPPSAIIILGSASQTENKNVTLSCVSKSSRPRVLLRWWLGWRQLLPMEETVMDGLHGGHISMSNLTFLARREDNGLTLTCEAFSEAFTKETFKKSLILNVKYPAQKLWIEGPPEGQKLRAGTRVRLVCLAIGGNPEPSLMWYKDSRTVTESRLPQESRRVHLGSVEKSGSTFSRELVLVTGPSDNQAKFTCKAGQLSASTQLAVQFPPTNVTILANASALRPGDALNLTCVSVSSNPPVNLSWDKEGERLEGVAAPPRRAPFKGSAAARSVLLQVSSRDHGQRVTCRAHSAELRETVSSFYRLNVLYRPEFLGEQVLVVTAVEQGEALLPVSVSANPAPEAFNWTFRGYRLSPAGGPRHRILSSGALHLWNVTRADDGLYQLHCQNSEGTAEARLRLDVHYAPTIRALQDPTEVNVGGSVDIVCTVDANPILPGMFNWERLGEDEEDQSLDDMEKISRGPTGRLRIHHAKLAQAGAYQCIVDNGVAPPARRLLRLVVRFAPQVEHPTPLTKVAAAGDSTSSATLHCRARGVPNIVFTWTKNGVPLDLQDPRYTEHTYHQGGVHSSLLTIANVSAAQDYALFTCTATNALGSDQTNIQLVSISRPDPPSGLKVVSLTPHSVGLEWKPGFDGGLPQRFCIRYEALGTPGFHYVDVVPPQATTFTLTGLQPSTRYRVWLLASNALGDSGLADKGTQLPITTPGLEGSGSGSHHHHHHHHGSGLNDIFEAQKIEWHE

SEQ ID NO: 90 - protein, 1070 aa, synthetic construct
MALGTTLRASLLLLGLLTEGLAQLAIPASVPRGFWALPENLTVVEGASVELRCGVSTPGSAVQWAKDGLLLGPDPRIPGFPRYRLEGDPARGEFHLHIEACDLSDDAEYECQVGRSEMGPELVSPRVILSILVPPKLLLLTPEAGTMVTWVAGQEYVVNCVSGDAKPAPDITILLSGQTISDISANVNEGSQQKLFTVEATARVTPRSSDNRQLLVCEASSPALAAPIKASATANVLFPPGPPVIEWPGLDEGHVRAGQSLELPCVARGGNPLATLQWLKNGQPVSTAWGTEHTQAVARSVLVMTVRPEDHGAQLSCEAHNSVSAGTQEHGITLQVTFPPSAIIILGSASQTENKNVTLSCVSKSSRPRVLLRWWLGWRQLLPMEETVMDGLHGGHISMSNLTFLARREDNGLTLTCEAFSEAFTKETFKKSLILNVKYPAQKLWIEGPPEGQKLRAGTRVRLVCLAIGGNPEPSLMWYKDSRTVTESRLPQESRRVHLGSVEKSGSTFSRELVLVTGPSDNQAKFTCKAGQLSASTQLAVQFPPTNVTILANASALRPGDALNLTCVSVSSNPPVNLSWDKEGERLEGVAAPPRRAPFKGSAAARSVLLQVSSRDHGQRVTCRAHSAELRETVSSFYRLNVLYRPEFLGEQVLVVTAVEQGEALLPVSVSANPAPEAFNWTFRGYRLSPAGGPRHRILSSGALHLWNVTRADDGLYQLHCQNSEGTAEARLRLDVHYAPTIRALQDPTEVNVGGSVDIVCTVDANPILPGMFNWERLGEDEEDQSLDDMEKISRGPTGRLRIHHAKLAQAGAYQCIVDNGVAPPARRLLRLVVRFAPQVEHPTPLTKVAAAGDSTSSATLHCRARGVPNIVFTWTKNGVPLDLQDPRYTEHTYHQGGVHSSLLTIANVSAAQDYALFTCTATNALGSDQTNIQLVSISRPDPPSGLKVVSLTPHSVGLEWKPGFDGGLPQRFCIRYEALGTPGFHYVDVVPPQATTFTLTGLQPSTRYRVWLLASNALGDSGLADKGTQLPITTPGLEGSGSGSHHHHHHHHGSGLNDIFEAQKIEWHE

SEQ ID NO: 91 - protein, 1070 aa, synthetic construct
MALGTTLRASLLLLGLLTEGLAQLAIPASVPRGFWALPENLTVVEGASVELRCGVSTPGSAVQWAKDGLLLGPDPRIPGFPRYRLEGDPARGEFHLHIEACDLSDDAEYECQVGRSEMGPELVSPRVILSILVPPKLLLLTPEAGTMVTWVAGQEYVVNCVSGDAKPAPDITILLSGQTISDISANVNEGSQQKLFTVEATARVTPRSSDNRQLLVCEASSPALVSPIKVSITMNVLFPPGPPVIEWPGLDEGHVRAGQSLELPCVARGGNPLATLQWLKNGQPVSTAWGTEHTQAVARSVLVMTVRPEDHGAQLSCEAHNSVSAGTQEHGITLQVTFPPSAIIILGSASQTENKNVTLSCVSKSSRPRVLLRWWLGWRQLLPMEETVMDGLHGGHISMSNLTFLARREDNGLTLTCEAFSEAFTKETFKKSLILNVKYPAQKLWIEGPPEGQKLRAGTRVRLVCLAIGGNPEPSLMWYKDSRTVTESRLPQESRRVHLGSVEKSGSTFSRELVLVTGPSDNQAKFTCKAGQLSASTQLAVQFPPTNVTILANASALRPGDALNLTCVSVSSNPPVNLSWDKEGERLEGVAAPPRRAPFKGSAAARSVLLQVSSRDHGQRVTCRAHSAELRETVSSFYRLNVLYRPEFLGEQVLVVTAVEQGEALLPVSVSANPAPEAFNWTFRGYRLSPAGGPRHRILSSGALHLWNVTRADDGLYQLHCQNSEGTAEARLRLDVHYAPTIRALQDPTEVNVGGSVDIVCTVDANPILPGMFNWERLGEDEEDQSLDDMEKISRGPTGRLRIHHAKLAQAGAYQCIVDNGVAPPARRLLRLVVRFAPQVEHPTPLTKVAAAGDSTSSATLHCRARGVPNIVFTWTKNGVPLDLQDPRYTEHTYHQGGVHSSLLTIANVSAAQDYALFTCTATNALGSDQTNIQLVSISRPDPPSGLKVVSLTPHSVGLEWKPGFDGGLPQRFCIRYEALGTPGFHYVDVVPPQATTFTLTGLQPSTRYRVWLLASNALGDSGLADKGTQLPITTPGLEGSGSGSHHHHHHHHGSGLNDIFEAQKIEWHE

SEQ ID NO: 92 - protein, 1070 aa, synthetic construct
MALGTTLRASLLLLGLLTEGLAQLAIPASVPRGFWALPENLTVVEGASVELRCGVSTPGSAVQWAKDGLLLGPDPRIPGFPRYRLEGDPARGEFHLHIEACDLSDDAEYECQVGRSEMGPELVSPRVILSILVPPKLLLLTPEAGTMVTWVAGQEYVVNCVSGDAKPAPDITILLSGQTISDISANVNEGSQQKLFTVEATARVTPRSSDNRQLLVCEASSPALEAPIKASFTVNVLFPPGPPVIEWPGLAEGHVRAGQSLELPCVARGGNPLATLQWLKNGQPVSTAWGTEHTQAVARSVLVMTVRPEDHGAQLSCEAHNSVSAGTQEHGITLQVTFPPSAIIILGSASQTENKNVTLSCVSKSSRPRVLLRWWLGWRQLLPMEETVMDGLHGGHISMSNLTFLARREDNGLTLTCEAFSEAFTKETFKKSLILNVKYPAQKLWIEGPPEGQKLRAGTRVRLVCLAIGGNPEPSLMWYKDSRTVTESRLPQESRRVHLGSVEKSGSTFSRELVLVTGPSDNQAKFTCKAGQLSASTQLAVQFPPTNVTILANASALRPGDALNLTCVSVSSNPPVNLSWDKEGERLEGVAAPPRRAPFKGSAAARSVLLQVSSRDHGQRVTCRAHSAELRETVSSFYRLNVLYRPEFLGEQVLVVTAVEQGEALLPVSVSANPAPEAFNWTFRGYRLSPAGGPRHRILSSGALHLWNVTRADDGLYQLHCQNSEGTAEARLRLDVHYAPTIRALQDPTEVNVGGSVDIVCTVDANPILPGMFNWERLGEDEEDQSLDDMEKISRGPTGRLRIHHAKLAQAGAYQCIVDNGVAPPARRLLRLVVRFAPQVEHPTPLTKVAAAGDSTSSATLHCRARGVPNIVFTWTKNGVPLDLQDPRYTEHTYHQGGVHSSLLTIANVSAAQDYALFTCTATNALGSDQTNIQLVSISRPDPPSGLKVVSLTPHSVGLEWKPGFDGGLPQRFCIRYEALGTPGFHYVDVVPPQATTFTLTGLQPSTRYRVWLLASNALGDSGLADKGTQLPITTPGLEGSGSGSHHHHHHHHGSGLNDIFEAQKIEWHE

SEQ ID NO: 93 - protein, 1070 aa, synthetic construct
MALGTTLRASLLLLGLLTEGLAQLAIPASVPRGFWALPENLTVVEGASVELRCGVSTPGSAVQWAKDGLLLGPDPRIPGFPRYRLEGDPARGEFHLHIEACDLSDDAEYECQVGRSEMGPELVSPRVILSILVPPKLLLLTPEAGTMVTWVAGQEYVVNCVSGDAKPAPDITILLSGQTISDISANVNEGSQQKLFTVEATARVTPRSSDNRQLLVCEASSPALEAPIKASFTVNVLFPPGPPVIEWPGLNEGHVRAGQSLELPCVARGGNPLATLQWLKNGQPVSTAWGTEHTQAVARSVLVMTVRPEDHGAQLSCEAHNSVSAGTQEHGITLQVTFPPSAIIILGSASQTENKNVTLSCVSKSSRPRVLLRWWLGWRQLLPMEETVMDGLHGGHISMSNLTFLARREDNGLTLTCEAFSEAFTKETFKKSLILNVKYPAQKLWIEGPPEGQKLRAGTRVRLVCLAIGGNPEPSLMWYKDSRTVTESRLPQESRRVHLGSVEKSGSTFSRELVLVTGPSDNQAKFTCKAGQLSASTQLAVQFPPTNVTILANASALRPGDALNLTCVSVSSNPPVNLSWDKEGERLEGVAAPPRRAPFKGSAAARSVLLQVSSRDHGQRVTCRAHSAELRETVSSFYRLNVLYRPEFLGEQVLVVTAVEQGEALLPVSVSANPAPEAFNWTFRGYRLSPAGGPRHRILSSGALHLWNVTRADDGLYQLHCQNSEGTAEARLRLDVHYAPTIRALQDPTEVNVGGSVDIVCTVDANPILPGMFNWERLGEDEEDQSLDDMEKISRGPTGRLRIHHAKLAQAGAYQCIVDNGVAPPARRLLRLVVRFAPQVEHPTPLTKVAAAGDSTSSATLHCRARGVPNIVFTWTKNGVPLDLQDPRYTEHTYHQGGVHSSLLTIANVSAAQDYALFTCTATNALGSDQTNIQLVSISRPDPPSGLKVVSLTPHSVGLEWKPGFDGGLPQRFCIRYEALGTPGFHYVDVVPPQATTFTLTGLQPSTRYRVWLLASNALGDSGLADKGTQLPITTPGLEGSGSGSHHHHHHHHGSGLNDIFEAQKIEWHE

SEQ ID NO: 94 - protein, 1070 aa, synthetic construct
MALGTTLRASLLLLGLLTEGLAQLAIPASVPRGFWALPENLTVVEGASVELRCGVSTPGSAVQWAKDGLLLGPDPRIPGFPRYRLEGDPARGEFHLHIEACDLSDDAEYECQVGRSEMGPELVSPRVILSILVPPKLLLLTPEAGTMVTWVAGQEYVVNCVSGDAKPAPDITILLSGQTISDISANVNEGSQQKLFTVEATARVTPRSSDNRQLLVCEASSPALEAPIKASFTVNVLFPPGPPVIEWPGLDEGHVRAGQSLELPCVARGGNPLATLQWLKNGQPVSTAWGTEHTQAVARSVLVMTVRPEDHGAQLSCEAHNSVSAGTQEHGITLQVTFPPSAIIILGSASQTENKNVTLSCVSKSSRPRVLLRWWLGWRQLLPMEETVMDGLHGGHISMSNLTFLARREDNGLTLTCEAFSEAFTKETFKKSLILNVKYPAQKLWIEGPPEGQALRAGTRVRLVCLAIGGNPEPSLMWYKDSRTVTESRLPQESRRVHLGSVEKSGSTFSRELVLVTGPSDNQAKFTCKAGQLSASTQLAVQFPPTNVTILANASALRPGDALNLTCVSVSSNPPVNLSWDKEGERLEGVAAPPRRAPFKGSAAARSVLLQVSSRDHGQRVTCRAHSAELRETVSSFYRLNVLYRPEFLGEQVLVVTAVEQGEALLPVSVSANPAPEAFNWTFRGYRLSPAGGPRHRILSSGALHLWNVTRADDGLYQLHCQNSEGTAEARLRLDVHYAPTIRALQDPTEVNVGGSVDIVCTVDANPILPGMFNWERLGEDEEDQSLDDMEKISRGPTGRLRIHHAKLAQAGAYQCIVDNGVAPPARRLLRLVVRFAPQVEHPTPLTKVAAAGDSTSSATLHCRARGVPNIVFTWTKNGVPLDLQDPRYTEHTYHQGGVHSSLLTIANVSAAQDYALFTCTATNALGSDQTNIQLVSISRPDPPSGLKVVSLTPHSVGLEWKPGFDGGLPQRFCIRYEALGTPGFHYVDVVPPQATTFTLTGLQPSTRYRVWLLASNALGDSGLADKGTQLPITTPGLEGSGSGSHHHHHHHHGSGLNDIFEAQKIEWHE

SEQ ID NO: 95 - protein, 1070 aa, synthetic construct
MALGTTLRASLLLLGLLTEGLAQLAIPASVPRGFWALPENLTVVEGASVELRCGVSTPGSAVQWAKDGLLLGPDPRIPGFPRYRLEGDPARGEFHLHIEACDLSDDAEYECQVGRSEMGPELVSPRVILSILVPPKLLLLTPEAGTMVTWVAGQEYVVNCVSGDAKPAPDITILLSGQTISDISANVNEGSQQKLFTVEATARVTPRSSDNRQLLVCEASSPALEAPIKASFTVNVLFPPGPPVIEWPGLDEGHVRAGQSLELPCVARGGNPLATLQWLKNGQPVSTAWGTEHTQAVARSVLVMTVRPEDHGAQLSCEAHNSVSAGTQEHGITLQVTFPPSAIIILGSASQTENKNVTLSCVSKSSRPRVLLRWWLGWRQLLPMEETVMDGLHGGHISMSNLTFLARREDNGLTLTCEAFSEAFTKETFKKSLILNVKYPAQKLWIEGPPEGQRLRAGTRVRLVCLAIGGNPEPSLMWYKDSRTVTESRLPQESRRVHLGSVEKSGSTFSRELVLVTGPSDNQAKFTCKAGQLSASTQLAVQFPPTNVTILANASALRPGDALNLTCVSVSSNPPVNLSWDKEGERLEGVAAPPRRAPFKGSAAARSVLLQVSSRDHGQRVTCRAHSAELRETVSSFYRLNVLYRPEFLGEQVLVVTAVEQGEALLPVSVSANPAPEAFNWTFRGYRLSPAGGPRHRILSSGALHLWNVTRADDGLYQLHCQNSEGTAEARLRLDVHYAPTIRALQDPTEVNVGGSVDIVCTVDANPILPGMFNWERLGEDEEDQSLDDMEKISRGPTGRLRIHHAKLAQAGAYQCIVDNGVAPPARRLLRLVVRFAPQVEHPTPLTKVAAAGDSTSSATLHCRARGVPNIVFTWTKNGVPLDLQDPRYTEHTYHQGGVHSSLLTIANVSAAQDYALFTCTATNALGSDQTNIQLVSISRPDPPSGLKVVSLTPHSVGLEWKPGFDGGLPQRFCIRYEALGTPGFHYVDVVPPQATTFTLTGLQPSTRYRVWLLASNALGDSGLADKGTQLPITTPGLEGSGSGSHHHHHHHHGSGLNDIFEAQKIEWHE

SEQ ID NO: 96 - protein, 1070 aa, synthetic construct
MALGTTLRASLLLLGLLTEGLAQLAIPASVPRGFWALPENLTVVEGASVELRCGVSTPGSAVQWAKDGLLLGPDPRIPGFPRYRLEGDPARGEFHLHIEACDLSDDAEYECQVGRSEMGPELVSPRVILSILVPPKLLLLTPEAGTMVTWVAGQEYVVNCVSGDAKPAPDITILLSGQTISDISANVNEGSQQKLFTVEATARVTPRSSDNRQLLVCEASSPALEAPIKASFTVNVLFPPGPPVIEWPGLDEGHVRAGQSLELPCVARGGNPLATLQWLKNGQPVSTAWGTEHTQAVARSVLVMTVRPEDHGAQLSCEAHNSVSAGTQEHGITLQVTFPPSAIIILGSASQTENKNVTLSCVSKSSRPRVLLRWWLGWRQLLPMEETVMDGLHGGHISMSNLTFLARREDNGLTLTCEAFSEAFTKETFKKSLILNVKYPAQKLWIEGPPEGQKLRAGTRVRLVCLAIGGNPEPSLAWYKDSRTVTESRLPQESRRVHLGSVEKSGSTFSRELVLVTGPSDNQAKFTCKAGQLSASTQLAVQFPPTNVTILANASALRPGDALNLTCVSVSSNPPVNLSWDKEGERLEGVAAPPRRAPFKGSAAARSVLLQVSSRDHGQRVTCRAHSAELRETVSSFYRLNVLYRPEFLGEQVLVVTAVEQGEALLPVSVSANPAPEAFNWTFRGYRLSPAGGPRHRILSSGALHLWNVTRADDGLYQLHCQNSEGTAEARLRLDVHYAPTIRALQDPTEVNVGGSVDIVCTVDANPILPGMFNWERLGEDEEDQSLDDMEKISRGPTGRLRIHHAKLAQAGAYQCIVDNGVAPPARRLLRLVVRFAPQVEHPTPLTKVAAAGDSTSSATLHCRARGVPNIVFTWTKNGVPLDLQDPRYTEHTYHQGGVHSSLLTIANVSAAQDYALFTCTATNALGSDQTNIQLVSISRPDPPSGLKVVSLTPHSVGLEWKPGFDGGLPQRFCIRYEALGTPGFHYVDVVPPQATTFTLTGLQPSTRYRVWLLASNALGDSGLADKGTQLPITTPGLEGSGSGSHHHHHHHHGSGLNDIFEAQKIEWHE

SEQ ID NO: 97 - protein, 1070 aa, synthetic construct
MALGTTLRASLLLLGLLTEGLAQLAIPASVPRGFWALPENLTVVEGASVELRCGVSTPGSAVQWAKDGLLLGPDPRIPGFPRYRLEGDPARGEFHLHIEACDLSDDAEYECQVGRSEMGPELVSPRVILSILVPPKLLLLTPEAGTMVTWVAGQEYVVNCVSGDAKPAPDITILLSGQTISDISANVNEGSQQKLFTVEATARVTPRSSDNRQLLVCEASSPALEAPIKASFTVNVLFPPGPPVIEWPGLDEGHVRAGQSLELPCVARGGNPLATLQWLKNGQPVSTAWGTEHTQAVARSVLVMTVRPEDHGAQLSCEAHNSVSAGTQEHGITLQVTFPPSAIIILGSASQTENKNVTLSCVSKSSRPRVLLRWWLGWRQLLPMEETVMDGLHGGHISMSNLTFLARREDNGLTLTCEAFSEAFTKETFKKSLILNVKYPAQKLWIEGPPEGQKLRAGTRVRLVCLAIGGNPEPSLTWYKDSRTVTESRLPQESRRVHLGSVEKSGSTFSRELVLVTGPSDNQAKFTCKAGQLSASTQLAVQFPPTNVTILANASALRPGDALNLTCVSVSSNPPVNLSWDKEGERLEGVAAPPRRAPFKGSAAARSVLLQVSSRDHGQRVTCRAHSAELRETVSSFYRLNVLYRPEFLGEQVLVVTAVEQGEALLPVSVSANPAPEAFNWTFRGYRLSPAGGPRHRILSSGALHLWNVTRADDGLYQLHCQNSEGTAEARLRLDVHYAPTIRALQDPTEVNVGGSVDIVCTVDANPILPGMFNWERLGEDEEDQSLDDMEKISRGPTGRLRIHHAKLAQAGAYQCIVDNGVAPPARRLLRLVVRFAPQVEHPTPLTKVAAAGDSTSSATLHCRARGVPNIVFTWTKNGVPLDLQDPRYTEHTYHQGGVHSSLLTIANVSAAQDYALFTCTATNALGSDQTNIQLVSISRPDPPSGLKVVSLTPHSVGLEWKPGFDGGLPQRFCIRYEALGTPGFHYVDVVPPQATTFTLTGLQPSTRYRVWLLASNALGDSGLADKGTQLPITTPGLEGSGSGSHHHHHHHHGSGLNDIFEAQKIEWHE

SEQ ID NO: 98 - protein, 1070 aa, synthetic construct
MALGTTLRASLLLLGLLTEGLAQLAIPASVPRGFWALPENLTVVEGASVELRCGVSTPGSAVQWAKDGLLLGPDPRIPGFPRYRLEGDPARGEFHLHIEACDLSDDAEYECQVGRSEMGPELVSPRVILSILVPPKLLLLTPEAGTMVTWVAGQEYVVNCVSGDAKPAPDITILLSGQTISDISANVNEGSQQKLFTVEATARVTPRSSDNRQLLVCEASSPALEAPIKASFTVNVLFPPGPPVIEWPGLDEGHVRAGQSLELPCVARGGNPLATLQWLKNGQPVSTAWGTEHTQAVARSVLVMTVRPEDHGAQLSCEAHNSVSAGTQEHGITLQVTFPPSAIIILGSASQTENKNVTLSCVSKSSRPRVLLRWWLGWRQLLPMEETVMDGLHGGHISMSNLTFLARREDNGLTLTCEAFSEAFTKETFKKSLILNVKYPAQKLWIEGPPEGQKLRAGTRVRLVCLAIGGNPEPSLMWYKDSRTVTESRLPQESRRVHLGSVEKSGSTFSRELVLVTGPSDNQAKFTCKAGQLSASTQLAVQFPPTNVTILANASALRPGDALNLTCVSVSSNPPVNLSWDKEGERLEGVAAPPRRAPFKGSAAARSVLLQVSSRDHGQRVTCRAHSAELRETVSSFYRLNVLYRPEFLGEQVLVVTAVEQGEALLPVSVSANPAPEAFNWTFRGYRLSPAGGPRHRILSSGALHLWNVTRADDGLYQLHCQNSEGTAEARLRLDVHYAPTIRALQDPTEVNVGGSVDIVCTVDANPILPGMFNWERLGEDEEDQSLDDMEKISRGPTGRLRIHHAKLAQAGAYQCIVDNGVAPPARRLLRLVVRFAPQVEHPTPLTKVAAAGDSTSSATLHCRARGVPNIVFTWTKNGVPLDLQDPRYTEHTYHQGGVHSSLLTIANVSAAQDYALFTCTATNALGSDQTNIQLVSISRPDPPSGLKVVSLTPHSVGLEWKPGFDGGLPQRFCIRYEALATPGFHYVDVVPPQATTFTLTGLQPSTRYRVWLLASNALGDSGLADKGTQLPITTPGLEGSGSGSHHHHHHHHGSGLNDIFEAQKIEWHE

SEQ ID NO: 99 - protein, 1070 aa, synthetic construct
MALGTTLRASLLLLGLLTEGLAQLAIPASVPRGFWALPENLTVVEGASVELRCGVSTPGSAVQWAKDGLLLGPDPRIPGFPRYRLEGDPARGEFHLHIEACDLSDDAEYECQVGRSEMGPELVSPRVILSILVPPKLLLLTPEAGTMVTWVAGQEYVVNCVSGDAKPAPDITILLSGQTISDISANVNEGSQQKLFTVEATARVTPRSSDNRQLLVCEASSPALEAPIKASFTVNVLFPPGPPVIEWPGLDEGHVRAGQSLELPCVARGGNPLATLQWLKNGQPVSTAWGTEHTQAVARSVLVMTVRPEDHGAQLSCEAHNSVSAGTQEHGITLQVTFPPSAIIILGSASQTENKNVTLSCVSKSSRPRVLLRWWLGWRQLLPMEETVMDGLHGGHISMSNLTFLARREDNGLTLTCEAFSEAFTKETFKKSLILNVKYPAQKLWIEGPPEGQKLRAGTRVRLVCLAIGGNPEPSLMWYKDSRTVTESRLPQESRRVHLGSVEKSGSTFSRELVLVTGPSDNQAKFTCKAGQLSASTQLAVQFPPTNVTILANASALRPGDALNLTCVSVSSNPPVNLSWDKEGERLEGVAAPPRRAPFKGSAAARSVLLQVSSRDHGQRVTCRAHSAELRETVSSFYRLNVLYRPEFLGEQVLVVTAVEQGEALLPVSVSANPAPEAFNWTFRGYRLSPAGGPRHRILSSGALHLWNVTRADDGLYQLHCQNSEGTAEARLRLDVHYAPTIRALQDPTEVNVGGSVDIVCTVDANPILPGMFNWERLGEDEEDQSLDDMEKISRGPTGRLRIHHAKLAQAGAYQCIVDNGVAPPARRLLRLVVRFAPQVEHPTPLTKVAAAGDSTSSATLHCRARGVPNIVFTWTKNGVPLDLQDPRYTEHTYHQGGVHSSLLTIANVSAAQDYALFTCTATNALGSDQTNIQLVSISRPDPPSGLKVVSLTPHSVGLEWKPGFDGGLPQRFCIRYEALDTPGFHYVDVVPPQATTFTLTGLQPSTRYRVWLLASNALGDSGLADKGTQLPITTPGLEGSGSGSHHHHHHHHGSGLNDIFEAQKIEWHE

SEQ ID NO: 100 - protein, 1070 aa, synthetic construct
MALGTTLRASLLLLGLLTEGLAQLAIPASVPRGFWALPENLTVVEGASVELRCGVSTPGSAVQWAKDGLLLGPDPRIPGFPRYRLEGDPARGEFHLHIEACDLSDDAEYECQVGRSEMGPELVSPRVILSILVPPKLLLLTPEAGTMVTWVAGQEYVVNCVSGDAKPAPDITILLSGQTISDISANVNEGSQQKLFTVEATARVTPRSSDNRQLLVCEASSPALEAPIKASFTVNVLFPPGPPVIEWPGLDEGHVRAGQSLELPCVARGGNPLATLQWLKNGQPVSTAWGTEHTQAVARSVLVMTVRPEDHGAQLSCEAHNSVSAGTQEHGITLQVTFPPSAIIILGSASQTENKNVTLSCVSKSSRPRVLLRWWLGWRQLLPMEETVMDGLHGGHISMSNLTFLARREDNGLTLTCEAFSEAFTKETFKKSLILNVKYPAQKLWIEGPPEGQKLRAGTRVRLVCLAIGGNPEPSLMWYKDSRTVTESRLPQESRRVHLGSVEKSGSTFSRELVLVTGPSDNQAKFTCKAGQLSASTQLAVQFPPTNVTILANASALRPGDALNLTCVSVSSNPPVNLSWDKEGERLEGVAAPPRRAPFKGSAAARSVLLQVSSRDHGQRVTCRAHSAELRETVSSFYRLNVLYRPEFLGEQVLVVTAVEQGEALLPVSVSANPAPEAFNWTFRGYRLSPAGGPRHRILSSGALHLWNVTRADDGLYQLHCQNSEGTAEARLRLDVHYAPTIRALQDPTEVNVGGSVDIVCTVDANPILPGMFNWERLGEDEEDQSLDDMEKISRGPTGRLRIHHAKLAQAGAYQCIVDNGVAPPARRLLRLVVRFAPQVEHPTPLTKVAAAGDSTSSATLHCRARGVPNIVFTWTKNGVPLDLQDPRYTEHTYHQGGVHSSLLTIANVSAAQDYALFTCTATNALGSDQTNIQLVSISRPDPPSGLKVVSLTPHSVGLEWKPGFDGGLPQRFCIRYEALGTPGFHYVDVVPAQATTFTLTGLQPSTRYRVWLLASNALGDSGLADKGTQLPITTPGLEGSGSGSHHHHHHHHGSGLNDIFEAQKIEWHE

SEQ ID NO: 101 - protein, 105 aa, synthetic construct
VPPKLLLLTPEAGTMVTWVAGQEYVVNCVSGDAKPAPDITILLSGQTISDISANVNEGSQQKLFTVEATARVTPRSSDNRQLLVCEASSPALEAPIKASFTVNVL

SEQ ID NO: 102 - protein, 100 aa, synthetic construct
FPPGPPVIEWPGLDEGHVRAGQSLELPCVARGGNPLATLQWLKNGQPVSTAWGTEHTQAVARSVLVMTVRPEDHGAQLSCEAHNSVSAGTQEHGITLQVT

SEQ ID NO: 103 - protein, 205 aa, synthetic construct
VPPKLLLLTPEAGTMVTWVAGQEYVVNCVSGDAKPAPDITILLSGQTISDISANVNEGSQQKLFTVEATARVTPRSSDNRQLLVCEASSPALEAPIKASFTVNVLFPPGPPVIEWPGLDEGHVRAGQSLELPCVARGGNPLATLQWLKNGQPVSTAWGTEHTQAVARSVLVMTVRPEDHGAQLSCEAHNSVSAGTQEHGITLQVT